European Patent Application EP 4 556 568 A1, published May 21, 2025. Title: Biocatalytical methods for producing ethylenediamine-N,N′-disuccinic acid. Applicant: BASF SE. The sequence listing filed with the application follows.

SEQUENCE LISTING (91 sequences)

SEQ ID NO: 1 - protein, 495 aa, Chelatococcus asaccharovorans
MSAHVADATRIGRASGAKAPEFQELYDFDAAALTLTSAVFPYDSKIHRAHVVMLAEQAILTRDEASRILHGLAAADERASIDASLRTYLPYEAALKGEIGPVAGKMHIGRSRNDLANAGKRMFLRDQLLRTIEAVIGLRHAVVDKAAGHLDTVMVVYTQRKEAQPITLGHYLMAISENLGKNLDRFRELYPRVNQCPLGAAATAGTGWPLDRDRTADLLGFDGLVVNSIEGVAGWDHVAEFAFDNAIFLSGLSRLASEIQLWSSDEYQMAELDASFAGTSSIMPQKKNPDSLERSRKAAFAAMGPLVGILTSLNGIEYQYSAARVELEPRSIDAMIAATHAMTGVVRTLHPNKEQMLRYAAENYATMTDLTDMLVRRVGIDYREAHEIVARVVMAAIDQGIKANRIGLDLVQQAAIAQTGQPIAVSADDIADALDPVQNVARRKGKGMPAPESVQTAIDDARLELRTDHAWLDSARQRLAAADAALATAVEAIRA

SEQ ID NO: 2 - protein, 502 aa, Chelativorans sp. BNC1
MNINVPDATRIGRATGAKAPEFQELYDFDAAALTLTSAVFPYDSQIHRAHVVMLTEQGILTVEESATILSGLAQVDELAATDGSLRTYLPYEAALKRTIGSVAGKMHIGRSRNDLANAGKRMFLRDQLLRTIEAVIGYREAVVHKAADHLDTVMVVYTQRKEAQPITLGHYLMAISENLAKNLDRYRELYARINLCPLGAAATAGTGWPLNRDRTSALLGFDGLVVNSIEGVAGWDHVAEHAFVNAVFLSGLSRLASEIQLWSTDEYQVAELDASFAGTSSIMPQKKNPDSLERSRKAAFAAMGPLVGILTSLNAIEYQYSAARVELEPRSIDALIAATHAMTGVVRTLHPNKERMRQYAAENYSTMTDLTDMLVRRVGIDYREAHEIVAHVVITAIEKGIKANKIGLDLVQEAAVAQTGAGINVSADDIKDALDPWQNVLRREGKGMPAPMSVKASIDDAMAELHKDRAWLANATQALANAKQTLADSVQQIIQTDRKYLR

SEQ ID NO: 3 - protein, 609 aa, Bradyrhizobium sp. SK17
MRSMIADRHPVSHHIDSAGGVCPPCEGHGADRAIWTDSRIAIVMQPCIKAIAPAGRSQHDPAEHRPSVSAPRAVRNPIRRASGPMTLLTARAVLTASCSLVLAAALATASTRAQQNPALNDGTRIGRSAVPKAPEFQELYDFDAAAKTLGDATFPYEVRVHRAHVVMLAEKGIVTRSDAATILRGLDTVDARAADDASLRTYLPYEAALIKSIGPVAGRMHTGRSRNDLANTVNRMFYRDQLNRTVEALIALRSAVVAKAADNLDTVMVVYTHRKEAQPITLGHYLMAISESLGKSIDRYEQLYARVNQSPLGAAASAGTSWPLDRERTAALLGFDGLVIDTIEGTAGWDHIAEFASDNAIYLSGLSRLASEIQLWSTDEYRSAELDPAFAGTSSIMPQKKNPDSLERTRQIAANSVGAVTSVLTSLNAAEYQHSVTRVPLEPRSLDAMIAATHAMTGVVRTLQPNKEQMLRYAAQNFSTMTDLADTIVRESGIDFREAHEIIARVVEAAINGGKTADQIDVAMIETAAQAQLGRTIQISAAAVRDALDPVRSVKLRNGIGGPAASSVAAMIKVSQAEISDEQSRLAARRQKIAAASAALAQAVAAAEH

SEQ ID NO: 4 - protein, 495 aa, Brevundimonas diminuta MR-E001
MTPHNPDATRIGRASGAKAPEFQELYDFEAAALTLTSAVFPYDSKIHRAHVVMLAEQDILTRDEAASILNGLAKADELAGKDAALRTYLPYEAALKREIGSVAGKMHIGRSRNDLANAGKRMFLRDQLLRTVEAVIALREAVVTKAADHLDTVMVVYTQRKEAQPITLGHYLMAISENLGKNLARYRELHPRINQCPLGAAATAGTGWPLDRDRTAALLGFHGLVVNSIEGVAGWDHVAEFAFDNAVFLSGLSRLASEIQLWSTDEYQMAELDSAFAGTSSIMPQKKNPDSLERSRKAAFAAMGPLVAILTSLNGIEYQYSAARVELEPRSIDALIAATHAMTGVVRTLHPNKEQMLRYAAENYATMTDLTDLLVRRIGIDYREAHEIVARVVMTAIERGIKANAIGLDLVQEAAVAQTGNRIEIGAADIADALDPVQNVARRKGRGMPAPESVRAAIAEARQELDADKAWLEDRRAGLADADAALEEAVAGITT

SEQ ID NO: 5 - protein, 525 aa, Bradyrhizobium elkanii
MTLLTARAVLTASCSLVLAAALATASTRAQQNPALNDGTRIGRSAVPKAPEFQELYDFDAAAKTLGDATFPYEVRVHRAHVVMLAEKGIVTRSDAATILRGLDTVDARAADDASLRTYLPYEAALIKTIGPVAGRMHTGRSRNDLANTVNRMFYRDQLNRTVEALIALRSAVVAKAADNLDTVMVVYTHRKEAQPITLGHYLMAISESLGKSIDRYEQLYARVNQSPLGAAASAGTSWPLDRERTAALLGFDGLVIDTIEGTAGWDHIAEFASDNAIYLSGLSRLASEIQLWSTDEYRSAELDPAFAGTSSIMPQKKNPDSLERTRQIAANSVGAVTSVLTSLNAAEYQHSVTRVPLEPRSLDAMIAATHAMTGVVRTLQPNKEQMLRYAAQNFSTMTDLADTIVRESGIDFREAHEIIARVVEAAINGGKTADQIDVAMIETAAQAQLGRTIQISAAAVRDALDPVRSVKLRNGIGGPAASSVAAMIKVSQAEISDEQSRLAARRQKIAAASAALAQAVAAAEH

SEQ ID NO: 6 - protein, 518 aa, Pandoraea norimbergensis
MNRTPFALRLVTAAVLCLSWAAHAQTPDASRIGRTSVPKAPGFQALYDFDSAAKTLPDATFPYEVRVHRAHVVMLAEKGIISRDDARKILTGLDTIDARARDDASLRTYLPYEAALVKEIGSVAGRMHTGRSRNDLANTVNRMFYRDQINRTVTALIALRTAVIDKAEDNIDTVMVVYTHRKEAQPITLGHYLMALSEALKKDIDRYEELYVRMNQSPLGAAASAGTGWPLDRERTASLLGFDSLVVDTIEGTAGWDHITEFAADNAIYLSDLGRLGSEIQLWTTDEYRLAELDSAYAGISSIMPQKKNPDSIERTRAIAANSVGALTSILVSLNGIEYQHSVARVALEPRSIDGMIAATRAMTGVVQSLHVNKAQMLRDAAKNYSTMTDLADAIVRDSGIDFRDAHEIVAKVVDSAIQANLSADQITVDMVRRAAEQQLGHTVRISEASVRDALDPVRNVARRDGIGGPAPASVKRMIAQARKELDQEQAHLSQRTSALSSAGQRLDVAVAGITGTN

SEQ ID NO: 7 - protein, 499 aa, Caballeronia pedi
MSNTQGVKDATRIGRSSVAKAPEFQELYDFDAAAKTLVDATFPYESDIHHAHVVMLAECDIIKRDEAAQILRGLEAVDAQAKENPSLRTYLPYEAALKKAVGAVGGKMHLGRSRNDLANAVKRMFLRDQLNRVIEAVIALRASVVAKAADHLDTVMVVYTQRKEAQPITLGHYLMAYAESLGKSLDRYEQLYARINQCPLGAAATAGTGWPLDRERTSALLGFDSLVVNTIEGVAGWDHIAEFAADNAIYMSSLSRLASEIQLWSTDEYRSAELDPAFAGTSSIMPQKKNPDSLERTRQAAFATMGPLVAILTSLNGIEYQYSAARVGLEPRSIDGMIAATHAMTGVVRTLQPNAAQMLRYAAENFATMTDLTDMLVRKTGLDYREAHEVIARVVNAALDQGKKANVIDLDLVQDAARAQLGHTLDISATDVRDALDPVQNVARRNGIGGPAPVAVQRTIDTAQRELDEQRACYDTRMRKLADASRERARAVASMTAGS

SEQ ID NO: 8 - protein, 498 aa, Paraburkholderia sartisoli
MSDKQGVVDATRIGRSSVAKAPEFQELYEFDAAAKTLVDATFPYESQIHRAHVVMLAESGILKTQEVAEILRGLAVVDERARSDPSLRTYLPYEAALKKVVGSVGGKMHLGRSRNDLANAVKRMFLRDQANRTIEALIGLRAAVIAKAADNLDTVMVVYTQRKEAQPITLAHYLMAYSEGLGKSIERYEQMYARINHCPLGAAATAGTGWPLNRERTSGLLGFDALVVNTIEGVAGWDHIAEFAANNAIYMSSLSRLASEIQLWSTDEYRVAELDPSFAGTSSIMPQKKNPDSLERTRQAAAAAMGPFVSIVTSLNAIEYQYSAARVGLEPRSIDGIMAATHAMTGVVRTLQPNKAQMLKYASENFATMTDLTDMLVRECGLDYREAHEVIARVVNAAIDARKTANQIDLDMVQAAAHAQLGHPLDISAAAIAAALDPVQNVGRRNGIGGPAPSSVQQMIDNDRKALAEEQARLEDRFARLKHSGTDLDDAVKRIAGL

SEQ ID NO: 9 - protein, 495 aa, synthetic construct
MTPHNPDATRIGRAKRAKAPEFQELYDFEAAALTLTSAVFPYDSKIHRAHVVMLAEQDILTRDEAASILNGLAKADELAGKDAALRTYLPYEAALKREIGSVAGKMHIGRSANDLRNRVNACSCVTALRTVEAVIALREAVVTKAADHLDTVMVVYTQRKEAQPITLGHYLMAISENLGKNLARYRELHPRINQCPLGAAATAGTGWPLDRDRTAALLGFHGLVVNSIEGVAGWDHVAEFAFDNAVFLSGLSRLASEIQLWSTDEYQMAELDSAFAGTSSIMPQKKNPDSLERSRKGAFAAMGPLVAILTSLNGIEYQYSAARVELEPRSIDALIAATHAMTGVVRTLHPNKEQDACAMRQENYATMTDLTDLLVRRIGIDYREAHEIVARVVMTAIERGIKANAIGLDLVQEAAVAQTGNRIEIGAADIADALDPVQNVARRKGRGMPAPESVRAAIAEARQELDADKAWLEDRRAGLADADAALEEAVAGITT

SEQ ID NO: 10 - protein, 495 aa, synthetic construct
MSAHVADATRIGRASGAKAPEFQELYDFDAAALTLTSAVFPYDSKIHRAHVVMLAEQAILTRDEASRILHGLAAADERASIDASLRTYLPYEAALKGEIGPVAGKMHIGRSRNDLANAGKRMFLRDQLLRTIEAVIGLRHAVVDKAAGHLDTVMVVYTQRKEAQPTTLGHYLMAISENLGKNLDRFRELYPRVNQCPLGAAATAGTGWPLDRDRTADLLGFDGLVVNSIEGVAGWDHVAEFAFDNAIFLSGLSRLASEIQLWSSDEYQMAELDASFAGTSSIMPQKKNPDSLERSRKAAFAAMGPLVGILTSLNGIEYQYSAARVELEPRSIDAMIAATHAMTGVVRTLHPNKEQMLRYAAENYATMTDLTDMLVRRVGIDYREAHEIVARVVMAAIDQGIKANRIGLDLVQQAAIAQTGQPIAVSADDIADALDPVQNVARRKGKGMPAPESVQTAIDDARLELRTDHAWLDSARQRLAAADAALATAVEAIRA

SEQ ID NO: 11 - protein, 495 aa, synthetic construct
MSAHVADATRIGRASGAKAPEFQELYDFDAAALTLTSAVFPYDSKIHRAHVVMLAEQAILTRDEASRILHGLAAADERASIDASLRTYLPYEAALKGEIGPVAGKMHIGRSRNDLANAGERMFLRDQLLRTIEAVIGLRHAVVDKAAGHLDTVMVVYTQRKEAQPITLGHYLMAISENLGKNLDRFRELYPRVNQCPLGAAATAGTGWPLDRDRTADLLGFDGLVVNSIEGVAGWDHVAEFAFDNAIFLSGLSRLASEIQLWSSDEYQMAELDASFAGTSSIMPQKKNPDSLERSRKAAFAAMGPLVGILTSLNGIEYQYSAARVELEPRSIDAMIAATHAMTGVVRTLHPNKEQMLRYAAENYATMTDLTDMLVRRVGIDYREAHEIVARVVMAAIDQGIKANRIGLDLVQQAAIAQTGQPIAVSADDIADALDPVQNVARRKGKGMPAPESVQTAIDDARLELRTDHAWLDSARQRLAAADAALATAVEAIRA

SEQ ID NO: 12 - protein, 495 aa, synthetic construct
MSAHVADATRIGRASGAKAPEFQELYDFDAAALTLTSAVFPYDSKIHRAHVVMLAEQAILTRDEASRILHGLAAADERASIDASLRTYLPYEAALKGEIGPVAGKMHIGRSRNDLANAGKRMFLRDQLLRTIEAVIGLRHAVVDKAAGHLDTVMVVYTQRKEAQPSTLGHYLMAISENLGKNLDRFRELYPRVNQCPLGAAATAGTGWPLDRDRTADLLGFDGLVVNSIEGVAGWDHVAEFAFDNAIFLSGLSRLASEIQLWSSDEYQMAELDASFAGTSSIMPQKKNPDSLERSRKAAFAAMGPLVGILTSLNGIEYQYSAARVELEPRSIDAMIAATHAMTGVVRTLHPNKEQMLRYAAENYATMTDLTDMLVRRVGIDYREAHEIVARVVMAAIDQGIKANRIGLDLVQQAAIAQTGQPIAVSADDIADALDPVQNVARRKGKGMPAPESVQTAIDDARLELRTDHAWLDSARQRLAAADAALATAVEAIRA

SEQ ID NO: 13 - protein, 495 aa, synthetic construct
MSAHVADATRIGRASGAKAPEFQELYDFDAAALTLTSAVFPYDSKIHRAHVVMLAEQAILTRDEASRILHGLAAADERASIDASLRTYLPYEAALKGEIGPVAGKMHIGRSRNDLANAGKRMFLRDQLLRTIEAVIGLRHAVVDKAAGHLDTVMVVYTQRKEAQPITLGHYLMAISENLGKNLDRFRELYPRVNQCPLGAAATAGTGWPLDRDRTADLLGFDGLVVNSIEGVAGWDHVAEFAFDNAIFLSGLSRLASEIQLWSSDEYQMAELDASFAGTSSIMPQKKNPDSLERSRKAAFAAMGPLVGILTSLNGIEYQYSAARVELEPRSIDAMIAATHAMTGVVRTLHPNKEQMLRYAAENYVTMTDLTDMLVRRVGIDYREAHEIVARVVMAAIDQGIKANRIGLDLVQQAAIAQTGQPIAVSADDIADALDPVQNVARRKGKGMPAPESVQTAIDDARLELRTDHAWLDSARQRLAAADAALATAVEAIRA

SEQ ID NO: 14 - protein, 495 aa, synthetic construct
MSAHVADATRIGRASGAKAPEFQELYDFDAAALTLTSAVFPYDSKIHRAHVVMLAEQAILTRDEASRILHGLAAADERASIDASLRTYLPYEAALKGEIGPVAGKMHIGRSRNDLANAGERMFLRDQLLRTIEAVIGLRHAVVDKAAGHLDTVMVVYTQRKEAQPSTLGHYLMAISENLGKNLDRFRELYPRVNQCPLGAAATAGTGWPLDRDRTADLLGFDGLVVNSIEGVAGWDHVAEFAFDNAIFLSGLSRLASEIQLWSSDEYQMAELDASFAGTSSIMPQKKNPDSLERSRKAAFAAMGPLVGILTSLNGIEYQYSAARVELEPRSIDAMIAATHAMTGVVRTLHPNKEQMLRYAAENYVTMTDLTDMLVRRVGIDYREAHEIVARVVMAAIDQGIKANRIGLDLVQQAAIAQTGQPIAVSADDIADALDPVQNVARRKGKGMPAPESVQTAIDDARLELRTDHAWLDSARQRLAAADAALATAVEAIRA

SEQ ID NO: 15 - protein, 495 aa, synthetic construct
MSAHVADATRIGRASGAKAPEFQELYDFDAAALTLTSAVFPYDSKIHRAHVVMLAEQAILTRDEASRILHGLAAADERASIDASLRTYLPYEAALKGEIGPVAGKMHIGRSRNDLANAGERMFLRDQLLRTIEAVIGLRHAVVDKAAGHLDTVMVVYTQRKEAQPTTLGHYLMAISENLGKNLDRFRELYPRVNQCPLGAAATAGTGWPLDRDRTADLLGFDGLVVNSIEGVAGWDHVAEFAFDNAIFLSGLSRLASEIQLWSSDEYQMAELDASFAGTSSIMPQKKNPDSLERSRKAAFAAMGPLVGILTSLNGIEYQYSAARVELEPRSIDAMIAATHAMTGVVRTLHPNKEQMLRYAAENYVTMTDLTDMLVRRVGIDYREAHEIVARVVMAAIDQGIKANRIGLDLVQQAAIAQTGQPIAVSADDIADALDPVQNVARRKGKGMPAPESVQTAIDDARLELRTDHAWLDSARQRLAAADAALATAVEAIRA

SEQ ID NO: 16 - protein, 502 aa, synthetic construct
MNINVPDATRIGRATGAKAPEFQELYDFDAAALTLTSAVFPYDSQIHRAHVVMLTEQGILTVEESATILSGLAQVDELAATDGSLRTYLPYEAALKRTIGSVAGKMHIGRSRNDLANAGKRMFLRDQLLRTIEAVIGYREAVVHKAADHLDTVMVVYTQRKEAQPSTLGHYLMAISENLAKNLDRYRELYARINLCPLGAAATAGTGWPLNRDRTSALLGFDGLVVNSIEGVAGWDHVAEHAFVNAVFLSGLSRLASEIQLWSTDEYQVAELDASFAGTSSIMPQKKNPDSLERSRKAAFAAMGPLVGILTSLNAIEYQYSAARVELEPRSIDALIAATHAMTGVVRTLHPNKERMRQYAAENYSTMTDLTDMLVRRVGIDYREAHEIVAHVVITAIEKGIKANKIGLDLVQEAAVAQTGAGINVSADDIKDALDPWQNVLRREGKGMPAPMSVKASIDDAMAELHKDRAWLANATQALANAKQTLADSVQQIIQTDRKYLR

SEQ ID NO: 17 - protein, 502 aa, synthetic construct
MNINVPDATRIGRATGAKAPEFQELYDFDAAALTLTSAVFPYDSQIHRAHVVMLTEQGILTVEESATILSGLAQVDELAATDGSLRTYLPYEAALKRTIGSVAGKMHIGRSRNDLANAGERMFLRDQLLRTIEAVIGYREAVVHKAADHLDTVMVVYTQRKEAQPSTLGHYLMAISENLAKNLDRYRELYARINLCPLGAAATAGTGWPLNRDRTSALLGFDGLVVNSIEGVAGWDHVAEHAFVNAVFLSGLSRLASEIQLWSTDEYQVAELDASFAGTSSIMPQKKNPDSLERSRKAAFAAMGPLVGILTSLNAIEYQYSAARVELEPRSIDALIAATHAMTGVVRTLHPNKERMRQYAAENYVTMTDLTDMLVRRVGIDYREAHEIVAHVVITAIEKGIKANKIGLDLVQEAAVAQTGAGINVSADDIKDALDPWQNVLRREGKGMPAPMSVKASIDDAMAELHKDRAWLANATQALANAKQTLADSVQQIIQTDRKYLR

SEQ ID NO: 18 - protein, 502 aa, synthetic construct
MNINVPDATRIGRATGAKAPEFQELYDFDAAALTLTSAVFPYDSQIHRAHVVMLTEQGILTVEESATILSGLAQVDELAATDGSLRTYLPYEAALKRTIGSVAGKMHIGRSRNDLANAGKRMFLRDQLLRTIEAVIGYREAVVHKAADHLDTVMVVYTQRKEAQPITLGHYLMAISENLAKNLDRYRELYARINLCPLGAAATAGTGWPLNRDRTSALLGFDGLVVNSIEGVAGWDHVAEHAFVNAVFLSGLSRLASEIQLWSTDEYQVAELDASFAGTSSIMPQKKNPDSLERSRKAAFAAMGPLVGILTSLNAIEYQYSAARVELEPRSIDALIAATHAMTGVVRTLHPNKERMRQYAAENYVTMTDLTDMLVRRVGIDYREAHEIVAHVVITAIEKGIKANKIGLDLVQEAAVAQTGAGINVSADDIKDALDPWQNVLRREGKGMPAPMSVKASIDDAMAELHKDRAWLANATQALANAKQTLADSVQQIIQTDRKYLR

SEQ ID NO: 19 - protein, 502 aa, synthetic construct
MNINVPDATRIGRATGAKAPEFQELYDFDAAALTLTSAVFPYDSQIHRAHVVMLTEQGILTVEESATILSGLAQVDELAATDGSLRTYLPYEAALKRTIGSVAGKMHIGRSRNDLANAGERMFLRDQLLRTIEAVIGYREAVVHKAADHLDTVMVVYTQRKEAQPTTLGHYLMAISENLAKNLDRYRELYARINLCPLGAAATAGTGWPLNRDRTSALLGFDGLVVNSIEGVAGWDHVAEHAFVNAVFLSGLSRLASEIQLWSTDEYQVAELDASFAGTSSIMPQKKNPDSLERSRKAAFAAMGPLVGILTSLNAIEYQYSAARVELEPRSIDALIAATHAMTGVVRTLHPNKERMRQYAAENYVTMTDLTDMLVRRVGIDYREAHEIVAHVVITAIEKGIKANKIGLDLVQEAAVAQTGAGINVSADDIKDALDPWQNVLRREGKGMPAPMSVKASIDDAMAELHKDRAWLANATQALANAKQTLADSVQQIIQTDRKYLR

SEQ ID NO: 20 - protein, 502 aa, synthetic construct
MNINVPDATRIGRATGAKAPEFQELYDFDAAALTLTSAVFPYDSQIHRAHVVMLTEQGILTVEESATILSGLAQVDELAATDGSLRTYLPYEAALKRTIGSVAGKMHIGRSRNDLANAGERMFLRDQLLRTIEAVIGYREAVVHKAADHLDTVMVVYTQRKEAQPITLGHYLMAISENLAKNLDRYRELYARINLCPLGAAATAGTGWPLNRDRTSALLGFDGLVVNSIEGVAGWDHVAEHAFVNAVFLSGLSRLASEIQLWSTDEYQVAELDASFAGTSSIMPQKKNPDSLERSRKAAFAAMGPLVGILTSLNAIEYQYSAARVELEPRSIDALIAATHAMTGVVRTLHPNKERMRQYAAENYSTMTDLTDMLVRRVGIDYREAHEIVAHVVITAIEKGIKANKIGLDLVQEAAVAQTGAGINVSADDIKDALDPWQNVLRREGKGMPAPMSVKASIDDAMAELHKDRAWLANATQALANAKQTLADSVQQIIQTDRKYLR

SEQ ID NO: 21 - protein, 502 aa, synthetic construct
MNINVPDATRIGRATGAKAPEFQELYDFDAAALTLTSAVFPYDSQIHRAHVVMLTEQGILTVEESATILSGLAQVDELAATDGSLRTYLPYEAALKRTIGSVAGKMHIGRSRNDLANAGKRMFLRDQLLRTIEAVIGYREAVVHKAADHLDTVMVVYTQRKEAQPTTLGHYLMAISENLAKNLDRYRELYARINLCPLGAAATAGTGWPLNRDRTSALLGFDGLVVNSIEGVAGWDHVAEHAFVNAVFLSGLSRLASEIQLWSTDEYQVAELDASFAGTSSIMPQKKNPDSLERSRKAAFAAMGPLVGILTSLNAIEYQYSAARVELEPRSIDALIAATHAMTGVVRTLHPNKERMRQYAAENYSTMTDLTDMLVRRVGIDYREAHEIVAHVVITAIEKGIKANKIGLDLVQEAAVAQTGAGINVSADDIKDALDPWQNVLRREGKGMPAPMSVKASIDDAMAELHKDRAWLANATQALANAKQTLADSVQQIIQTDRKYLR

SEQ ID NO: 22 - protein, 495 aa, synthetic construct
MSAHVAMATRIGRASGAKAPEFQELYDFDAAALTLTSAVFPYDSKIHRAHVVMLAEQAILTRDEASRILHGLAAADERASIDASLRTYLPYEAALKGEIGPVAGKMHIGRSRNDLANAGKRMFLRDQLLRTIEAVIGLRHAVVDKAAGHLDTVMVVYTQRKEAQPITLGHYLMAISENLGKNLDRFRELYPRVNQCPLGAAATAGTGWPLDRDRTADLLGFDGLVVNSIEGVAGWDHVAEFAFDNAIFLSGLSRLASEIQLWSSDEYQMAELDASFAGTSSIMPQKKNPDSLERSRKAAFAAMGPLVGILTSLNGIEYQYSAARVELEPRSIDAMIAATHAMTGVVRTLHPNKEQMLRYAAENYATMTDLTDMLVRRVGIDYREAHEIVARVVMAAIDQGIKANRIGLDLVQQAAIAQTGQPIAVSADDIADALDPVQNVARRKGKGMPAPESVQTAIDDARLELRTDHAWLDSARQRLAAADAALATAVEAIRA

SEQ ID NO: 23 - protein, 495 aa, synthetic construct
MSAHVADALRIGRASGAKAPEFQELYDFDAAALTLTSAVFPYDSKIHRAHVVMLAEQAILTRDEASRILHGLAAADERASIDASLRTYLPYEAALKGEIGPVAGKMHIGRSRNDLANAGKRMFLRDQLLRTIEAVIGLRHAVVDKAAGHLDTVMVVYTQRKEAQPITLGHYLMAISENLGKNLDRFRELYPRVNQCPLGAAATAGTGWPLDRDRTADLLGFDGLVVNSIEGVAGWDHVAEFAFDNAIFLSGLSRLASEIQLWSSDEYQMAELDASFAGTSSIMPQKKNPDSLERSRKAAFAAMGPLVGILTSLNGIEYQYSAARVELEPRSIDAMIAATHAMTGVVRTLHPNKEQMLRYAAENYATMTDLTDMLVRRVGIDYREAHEIVARVVMAAIDQGIKANRIGLDLVQQAAIAQTGQPIAVSADDIADALDPVQNVARRKGKGMPAPESVQTAIDDARLELRTDHAWLDSARQRLAAADAALATAVEAIRA

SEQ ID NO: 24 - protein, 495 aa, synthetic construct
MSAHVADATWIGRASGAKAPEFQELYDFDAAALTLTSAVFPYDSKIHRAHVVMLAEQAILTRDEASRILHGLAAADERASIDASLRTYLPYEAALKGEIGPVAGKMHIGRSRNDLANAGKRMFLRDQLLRTIEAVIGLRHAVVDKAAGHLDTVMVVYTQRKEAQPITLGHYLMAISENLGKNLDRFRELYPRVNQCPLGAAATAGTGWPLDRDRTADLLGFDGLVVNSIEGVAGWDHVAEFAFDNAIFLSGLSRLASEIQLWSSDEYQMAELDASFAGTSSIMPQKKNPDSLERSRKAAFAAMGPLVGILTSLNGIEYQYSAARVELEPRSIDAMIAATHAMTGVVRTLHPNKEQMLRYAAENYATMTDLTDMLVRRVGIDYREAHEIVARVVMAAIDQGIKANRIGLDLVQQAAIAQTGQPIAVSADDIADALDPVQNVARRKGKGMPAPESVQTAIDDARLELRTDHAWLDSARQRLAAADAALATAVEAIRA

SEQ ID NO: 25 - protein, 495 aa, synthetic construct
MSAHVADATRIGRASGATAPEFQELYDFDAAALTLTSAVFPYDSKIHRAHVVMLAEQAILTRDEASRILHGLAAADERASIDASLRTYLPYEAALKGEIGPVAGKMHIGRSRNDLANAGKRMFLRDQLLRTIEAVIGLRHAVVDKAAGHLDTVMVVYTQRKEAQPITLGHYLMAISENLGKNLDRFRELYPRVNQCPLGAAATAGTGWPLDRDRTADLLGFDGLVVNSIEGVAGWDHVAEFAFDNAIFLSGLSRLASEIQLWSSDEYQMAELDASFAGTSSIMPQKKNPDSLERSRKAAFAAMGPLVGILTSLNGIEYQYSAARVELEPRSIDAMIAATHAMTGVVRTLHPNKEQMLRYAAENYATMTDLTDMLVRRVGIDYREAHEIVARVVMAAIDQGIKANRIGLDLVQQAAIAQTGQPIAVSADDIADALDPVQNVARRKGKGMPAPESVQTAIDDARLELRTDHAWLDSARQRLAAADAALATAVEAIRA

SEQ ID NO: 26 - protein, 495 aa, synthetic construct
MSAHVADATRIGRASGAKAPEFAELYDFDAAALTLTSAVFPYDSKIHRAHVVMLAEQAILTRDEASRILHGLAAADERASIDASLRTYLPYEAALKGEIGPVAGKMHIGRSRNDLANAGKRMFLRDQLLRTIEAVIGLRHAVVDKAAGHLDTVMVVYTQRKEAQPITLGHYLMAISENLGKNLDRFRELYPRVNQCPLGAAATAGTGWPLDRDRTADLLGFDGLVVNSIEGVAGWDHVAEFAFDNAIFLSGLSRLASEIQLWSSDEYQMAELDASFAGTSSIMPQKKNPDSLERSRKAAFAAMGPLVGILTSLNGIEYQYSAARVELEPRSIDAMIAATHAMTGVVRTLHPNKEQMLRYAAENYATMTDLTDMLVRRVGIDYREAHEIVARVVMAAIDQGIKANRIGLDLVQQAAIAQTGQPIAVSADDIADALDPVQNVARRKGKGMPAPESVQTAIDDARLELRTDHAWLDSARQRLAAADAALATAVEAIRA

SEQ ID NO: 27 - protein, 495 aa, synthetic construct
MSAHVADATRIGRASGAKAPEFQELDDFDAAALTLTSAVFPYDSKIHRAHVVMLAEQAILTRDEASRILHGLAAADERASIDASLRTYLPYEAALKGEIGPVAGKMHIGRSRNDLANAGKRMFLRDQLLRTIEAVIGLRHAVVDKAAGHLDTVMVVYTQRKEAQPITLGHYLMAISENLGKNLDRFRELYPRVNQCPLGAAATAGTGWPLDRDRTADLLGFDGLVVNSIEGVAGWDHVAEFAFDNAIFLSGLSRLASEIQLWSSDEYQMAELDASFAGTSSIMPQKKNPDSLERSRKAAFAAMGPLVGILTSLNGIEYQYSAARVELEPRSIDAMIAATHAMTGVVRTLHPNKEQMLRYAAENYATMTDLTDMLVRRVGIDYREAHEIVARVVMAAIDQGIKANRIGLDLVQQAAIAQTGQPIAVSADDIADALDPVQNVARRKGKGMPAPESVQTAIDDARLELRTDHAWLDSARQRLAAADAALATAVEAIRA

SEQ ID NO: 28 - protein, 495 aa, synthetic construct
MSAHVADATRIGRASGAKAPEFQELYEFDAAALTLTSAVFPYDSKIHRAHVVMLAEQAILTRDEASRILHGLAAADERASIDASLRTYLPYEAALKGEIGPVAGKMHIGRSRNDLANAGKRMFLRDQLLRTIEAVIGLRHAVVDKAAGHLDTVMVVYTQRKEAQPITLGHYLMAISENLGKNLDRFRELYPRVNQCPLGAAATAGTGWPLDRDRTADLLGFDGLVVNSIEGVAGWDHVAEFAFDNAIFLSGLSRLASEIQLWSSDEYQMAELDASFAGTSSIMPQKKNPDSLERSRKAAFAAMGPLVGILTSLNGIEYQYSAARVELEPRSIDAMIAATHAMTGVVRTLHPNKEQMLRYAAENYATMTDLTDMLVRRVGIDYREAHEIVARVVMAAIDQGIKANRIGLDLVQQAAIAQTGQPIAVSADDIADALDPVQNVARRKGKGMPAPESVQTAIDDARLELRTDHAWLDSARQRLAAADAALATAVEAIRA

SEQ ID NO: 29 - protein, 495 aa, synthetic construct
MSAHVADATRIGRASGAKAPEFQELYDFGAAALTLTSAVFPYDSKIHRAHVVMLAEQAILTRDEASRILHGLAAADERASIDASLRTYLPYEAALKGEIGPVAGKMHIGRSRNDLANAGKRMFLRDQLLRTIEAVIGLRHAVVDKAAGHLDTVMVVYTQRKEAQPITLGHYLMAISENLGKNLDRFRELYPRVNQCPLGAAATAGTGWPLDRDRTADLLGFDGLVVNSIEGVAGWDHVAEFAFDNAIFLSGLSRLASEIQLWSSDEYQMAELDASFAGTSSIMPQKKNPDSLERSRKAAFAAMGPLVGILTSLNGIEYQYSAARVELEPRSIDAMIAATHAMTGVVRTLHPNKEQMLRYAAENYATMTDLTDMLVRRVGIDYREAHEIVARVVMAAIDQGIKANRIGLDLVQQAAIAQTGQPIAVSADDIADALDPVQNVARRKGKGMPAPESVQTAIDDARLELRTDHAWLDSARQRLAAADAALATAVEAIRA

SEQ ID NO: 30 - protein, 495 aa, synthetic construct
MSAHVADATRIGRASGAKAPEFQELYDFDSAALTLTSAVFPYDSKIHRAHVVMLAEQAILTRDEASRILHGLAAADERASIDASLRTYLPYEAALKGEIGPVAGKMHIGRSRNDLANAGKRMFLRDQLLRTIEAVIGLRHAVVDKAAGHLDTVMVVYTQRKEAQPITLGHYLMAISENLGKNLDRFRELYPRVNQCPLGAAATAGTGWPLDRDRTADLLGFDGLVVNSIEGVAGWDHVAEFAFDNAIFLSGLSRLASEIQLWSSDEYQMAELDASFAGTSSIMPQKKNPDSLERSRKAAFAAMGPLVGILTSLNGIEYQYSAARVELEPRSIDAMIAATHAMTGVVRTLHPNKEQMLRYAAENYATMTDLTDMLVRRVGIDYREAHEIVARVVMAAIDQGIKANRIGLDLVQQAAIAQTGQPIAVSADDIADALDPVQNVARRKGKGMPAPESVQTAIDDARLELRTDHAWLDSARQRLAAADAALATAVEAIRA

SEQ ID NO: 31 - protein, 495 aa, synthetic construct
MSAHVADATRIGRASGAKAPEFQELYDFDAAALTLTDAVFPYDSKIHRAHVVMLAEQAILTRDEASRILHGLAAADERASIDASLRTYLPYEAALKGEIGPVAGKMHIGRSRNDLANAGKRMFLRDQLLRTIEAVIGLRHAVVDKAAGHLDTVMVVYTQRKEAQPITLGHYLMAISENLGKNLDRFRELYPRVNQCPLGAAATAGTGWPLDRDRTADLLGFDGLVVNSIEGVAGWDHVAEFAFDNAIFLSGLSRLASEIQLWSSDEYQMAELDASFAGTSSIMPQKKNPDSLERSRKAAFAAMGPLVGILTSLNGIEYQYSAARVELEPRSIDAMIAATHAMTGVVRTLHPNKEQMLRYAAENYATMTDLTDMLVRRVGIDYREAHEIVARVVMAAIDQGIKANRIGLDLVQQAAIAQTGQPIAVSADDIADALDPVQNVARRKGKGMPAPESVQTAIDDARLELRTDHAWLDSARQRLAAADAALATAVEAIRA

SEQ ID NO: 32 - protein, 495 aa, synthetic construct
MSAHVADATRIGRASGAKAPEFQELYDFDAAALTLTSEVFPYDSKIHRAHVVMLAEQAILTRDEASRILHGLAAADERASIDASLRTYLPYEAALKGEIGPVAGKMHIGRSRNDLANAGKRMFLRDQLLRTIEAVIGLRHAVVDKAAGHLDTVMVVYTQRKEAQPITLGHYLMAISENLGKNLDRFRELYPRVNQCPLGAAATAGTGWPLDRDRTADLLGFDGLVVNSIEGVAGWDHVAEFAFDNAIFLSGLSRLASEIQLWSSDEYQMAELDASFAGTSSIMPQKKNPDSLERSRKAAFAAMGPLVGILTSLNGIEYQYSAARVELEPRSIDAMIAATHAMTGVVRTLHPNKEQMLRYAAENYATMTDLTDMLVRRVGIDYREAHEIVARVVMAAIDQGIKANRIGLDLVQQAAIAQTGQPIAVSADDIADALDPVQNVARRKGKGMPAPESVQTAIDDARLELRTDHAWLDSARQRLAAADAALATAVEAIRA

SEQ ID NO: 33 - protein, 495 aa, synthetic construct
MSAHVADATRIGRASGAKAPEFQELYDFDAAALTLTSATFPYDSKIHRAHVVMLAEQAILTRDEASRILHGLAAADERASIDASLRTYLPYEAALKGEIGPVAGKMHIGRSRNDLANAGKRMFLRDQLLRTIEAVIGLRHAVVDKAAGHLDTVMVVYTQRKEAQPITLGHYLMAISENLGKNLDRFRELYPRVNQCPLGAAATAGTGWPLDRDRTADLLGFDGLVVNSIEGVAGWDHVAEFAFDNAIFLSGLSRLASEIQLWSSDEYQMAELDASFAGTSSIMPQKKNPDSLERSRKAAFAAMGPLVGILTSLNGIEYQYSAARVELEPRSIDAMIAATHAMTGVVRTLHPNKEQMLRYAAENYATMTDLTDMLVRRVGIDYREAHEIVARVVMAAIDQGIKANRIGLDLVQQAAIAQTGQPIAVSADDIADALDPVQNVARRKGKGMPAPESVQTAIDDARLELRTDHAWLDSARQRLAAADAALATAVEAIRA

SEQ ID NO: 34 - protein, 495 aa, synthetic construct
MSAHVADATRIGRASGAKAPEFQELYDFDAAALTLTSAVFPYDSKIHRAHVVMLAEQGILTRDEASRILHGLAAADERASIDASLRTYLPYEAALKGEIGPVAGKMHIGRSRNDLANAGKRMFLRDQLLRTIEAVIGLRHAVVDKAAGHLDTVMVVYTQRKEAQPITLGHYLMAISENLGKNLDRFRELYPRVNQCPLGAAATAGTGWPLDRDRTADLLGFDGLVVNSIEGVAGWDHVAEFAFDNAIFLSGLSRLASEIQLWSSDEYQMAELDASFAGTSSIMPQKKNPDSLERSRKAAFAAMGPLVGILTSLNGIEYQYSAARVELEPRSIDAMIAATHAMTGVVRTLHPNKEQMLRYAAENYATMTDLTDMLVRRVGIDYREAHEIVARVVMAAIDQGIKANRIGLDLVQQAAIAQTGQPIAVSADDIADALDPVQNVARRKGKGMPAPESVQTAIDDARLELRTDHAWLDSARQRLAAADAALATAVEAIRA

SEQ ID NO: 35 - protein, 495 aa, synthetic construct
MSAHVADATRIGRASGAKAPEFQELYDFDAAALTLTSAVFPYDSKIHRAHVVMLAEQAILTRDEASRILHGLAAADERASIDASLDTYLPYEAALKGEIGPVAGKMHIGRSRNDLANAGKRMFLRDQLLRTIEAVIGLRHAVVDKAAGHLDTVMVVYTQRKEAQPITLGHYLMAISENLGKNLDRFRELYPRVNQCPLGAAATAGTGWPLDRDRTADLLGFDGLVVNSIEGVAGWDHVAEFAFDNAIFLSGLSRLASEIQLWSSDEYQMAELDASFAGTSSIMPQKKNPDSLERSRKAAFAAMGPLVGILTSLNGIEYQYSAARVELEPRSIDAMIAATHAMTGVVRTLHPNKEQMLRYAAENYATMTDLTDMLVRRVGIDYREAHEIVARVVMAAIDQGIKANRIGLDLVQQAAIAQTGQPIAVSADDIADALDPVQNVARRKGKGMPAPESVQTAIDDARLELRTDHAWLDSARQRLAAADAALATAVEAIRA

SEQ ID NO: 36 - protein, 495 aa, synthetic construct
MSAHVADATRIGRASGAKAPEFQELYDFDAAALTLTSAVFPYDSKIHRAHVVMLAEQAILTRDEASRILHGLAAADERASIDASLRVYLPYEAALKGEIGPVAGKMHIGRSRNDLANAGKRMFLRDQLLRTIEAVIGLRHAVVDKAAGHLDTVMVVYTQRKEAQPITLGHYLMAISENLGKNLDRFRELYPRVNQCPLGAAATAGTGWPLDRDRTADLLGFDGLVVNSIEGVAGWDHVAEFAFDNAIFLSGLSRLASEIQLWSSDEYQMAELDASFAGTSSIMPQKKNPDSLERSRKAAFAAMGPLVGILTSLNGIEYQYSAARVELEPRSIDAMIAATHAMTGVVRTLHPNKEQMLRYAAENYATMTDLTDMLVRRVGIDYREAHEIVARVVMAAIDQGIKANRIGLDLVQQAAIAQTGQPIAVSADDIADALDPVQNVARRKGKGMPAPESVQTAIDDARLELRTDHAWLDSARQRLAAADAALATAVEAIRA

SEQ ID NO: 37 - protein, 495 aa, synthetic construct
MSAHVADATRIGRASGAKAPEFQELYDFDAAALTLTSAVFPYDSKIHRAHVVMLAEQAILTRDEASRILHGLAAADERASIDASLRTYMPYEAALKGEIGPVAGKMHIGRSRNDLANAGKRMFLRDQLLRTIEAVIGLRHAVVDKAAGHLDTVMVVYTQRKEAQPITLGHYLMAISENLGKNLDRFRELYPRVNQCPLGAAATAGTGWPLDRDRTADLLGFDGLVVNSIEGVAGWDHVAEFAFDNAIFLSGLSRLASEIQLWSSDEYQMAELDASFAGTSSIMPQKKNPDSLERSRKAAFAAMGPLVGILTSLNGIEYQYSAARVELEPRSIDAMIAATHAMTGVVRTLHPNKEQMLRYAAENYATMTDLTDMLVRRVGIDYREAHEIVARVVMAAIDQGIKANRIGLDLVQQAAIAQTGQPIAVSADDIADALDPVQNVARRKGKGMPAPESVQTAIDDARLELRTDHAWLDSARQRLAAADAALATAVEAIRA

SEQ ID NO: 38 - protein, 495 aa, synthetic construct
MSAHVADATRIGRASGAKAPEFQELYDFDAAALTLTSAVFPYDSKIHRAHVVMLAEQAILTRDEASRILHGLAAADERASIDASLRTYLAYEAALKGEIGPVAGKMHIGRSRNDLANAGKRMFLRDQLLRTIEAVIGLRHAVVDKAAGHLDTVMVVYTQRKEAQPITLGHYLMAISENLGKNLDRFRELYPRVNQCPLGAAATAGTGWPLDRDRTADLLGFDGLVVNSIEGVAGWDHVAEFAFDNAIFLSGLSRLASEIQLWSSDEYQMAELDASFAGTSSIMPQKKNPDSLERSRKAAFAAMGPLVGILTSLNGIEYQYSAARVELEPRSIDAMIAATHAMTGVVRTLHPNKEQMLRYAAENYATMTDLTDMLVRRVGIDYREAHEIVARVVMAAIDQGIKANRIGLDLVQQAAIAQTGQPIAVSADDIADALDPVQNVARRKGKGMPAPESVQTAIDDARLELRTDHAWLDSARQRLAAADAALATAVEAIRA

SEQ ID NO: 39 - protein, 495 aa, synthetic construct
MSAHVADATRIGRASGAKAPEFQELYDFDAAALTLTSAVFPYDSKIHRAHVVMLAEQAILTRDEASRILHGLAAADERASIDASLRTYLPIEAALKGEIGPVAGKMHIGRSRNDLANAGKRMFLRDQLLRTIEAVIGLRHAVVDKAAGHLDTVMVVYTQRKEAQPITLGHYLMAISENLGKNLDRFRELYPRVNQCPLGAAATAGTGWPLDRDRTADLLGFDGLVVNSIEGVAGWDHVAEFAFDNAIFLSGLSRLASEIQLWSSDEYQMAELDASFAGTSSIMPQKKNPDSLERSRKAAFAAMGPLVGILTSLNGIEYQYSAARVELEPRSIDAMIAATHAMTGVVRTLHPNKEQMLRYAAENYATMTDLTDMLVRRVGIDYREAHEIVARVVMAAIDQGIKANRIGLDLVQQAAIAQTGQPIAVSADDIADALDPVQNVARRKGKGMPAPESVQTAIDDARLELRTDHAWLDSARQRLAAADAALATAVEAIRA

SEQ ID NO: 40 - protein, 495 aa, synthetic construct
MSAHVADATRIGRASGAKAPEFQELYDFDAAALTLTSAVFPYDSKIHRAHVVMLAEQAILTRDEASRILHGLAAADERASIDASLRTYLPYEAALIGEIGPVAGKMHIGRSRNDLANAGKRMFLRDQLLRTIEAVIGLRHAVVDKAAGHLDTVMVVYTQRKEAQPITLGHYLMAISENLGKNLDRFRELYPRVNQCPLGAAATAGTGWPLDRDRTADLLGFDGLVVNSIEGVAGWDHVAEFAFDNAIFLSGLSRLASEIQLWSSDEYQMAELDASFAGTSSIMPQKKNPDSLERSRKAAFAAMGPLVGILTSLNGIEYQYSAARVELEPRSIDAMIAATHAMTGVVRTLHPNKEQMLRYAAENYATMTDLTDMLVRRVGIDYREAHEIVARVVMAAIDQGIKANRIGLDLVQQAAIAQTGQPIAVSADDIADALDPVQNVARRKGKGMPAPESVQTAIDDARLELRTDHAWLDSARQRLAAADAALATAVEAIRA

SEQ ID NO: 41 - protein, 495 aa, synthetic construct
MSAHVADATRIGRASGAKAPEFQELYDFDAAALTLTSAVFPYDSKIHRAHVVMLAEQAILTRDEASRILHGLAAADERASIDASLRTYLPYEAALKGEIGPVAGKMHIGRSRNDMANAGKRMFLRDQLLRTIEAVIGLRHAVVDKAAGHLDTVMVVYTQRKEAQPITLGHYLMAISENLGKNLDRFRELYPRVNQCPLGAAATAGTGWPLDRDRTADLLGFDGLVVNSIEGVAGWDHVAEFAFDNAIFLSGLSRLASEIQLWSSDEYQMAELDASFAGTSSIMPQKKNPDSLERSRKAAFAAMGPLVGILTSLNGIEYQYSAARVELEPRSIDAMIAATHAMTGVVRTLHPNKEQMLRYAAENYATMTDLTDMLVRRVGIDYREAHEIVARVVMAAIDQGIKANRIGLDLVQQAAIAQTGQPIAVSADDIADALDPVQNVARRKGKGMPAPESVQTAIDDARLELRTDHAWLDSARQRLAAADAALATAVEAIRA

SEQ ID NO: 42 - protein, 495 aa, synthetic construct
MSAHVADATRIGRASGAKAPEFQELYDFDAAALTLTSAVFPYDSKIHRAHVVMLAEQAILTRDEASRILHGLAAADERASIDASLRTYLPYEAALKGEIGPVAGKMHIGRSRNDLVNAGKRMFLRDQLLRTIEAVIGLRHAVVDKAAGHLDTVMVVYTQRKEAQPITLGHYLMAISENLGKNLDRFRELYPRVNQCPLGAAATAGTGWPLDRDRTADLLGFDGLVVNSIEGVAGWDHVAEFAFDNAIFLSGLSRLASEIQLWSSDEYQMAELDASFAGTSSIMPQKKNPDSLERSRKAAFAAMGPLVGILTSLNGIEYQYSAARVELEPRSIDAMIAATHAMTGVVRTLHPNKEQMLRYAAENYATMTDLTDMLVRRVGIDYREAHEIVARVVMAAIDQGIKANRIGLDLVQQAAIAQTGQPIAVSADDIADALDPVQNVARRKGKGMPAPESVQTAIDDARLELRTDHAWLDSARQRLAAADAALATAVEAIRA

SEQ ID NO: 43 - protein, 495 aa, synthetic construct
MSAHVADATRIGRASGAKAPEFQELYDFDAAALTLTSAVFPYDSKIHRAHVVMLAEQAILTRDEASRILHGLAAADERASIDASLRTYLPYEAALKGEIGPVAGKMHIGRSRNDLANADKRMFLRDQLLRTIEAVIGLRHAVVDKAAGHLDTVMVVYTQRKEAQPITLGHYLMAISENLGKNLDRFRELYPRVNQCPLGAAATAGTGWPLDRDRTADLLGFDGLVVNSIEGVAGWDHVAEFAFDNAIFLSGLSRLASEIQLWSSDEYQMAELDASFAGTSSIMPQKKNPDSLERSRKAAFAAMGPLVGILTSLNGIEYQYSAARVELEPRSIDAMIAATHAMTGVVRTLHPNKEQMLRYAAENYATMTDLTDMLVRRVGIDYREAHEIVARVVMAAIDQGIKANRIGLDLVQQAAIAQTGQPIAVSADDIADALDPVQNVARRKGKGMPAPESVQTAIDDARLELRTDHAWLDSARQRLAAADAALATAVEAIRA

SEQ ID NO: 44 - protein, 495 aa, synthetic construct
MSAHVADATRIGRASGAKAPEFQELYDFDAAALTLTSAVFPYDSKIHRAHVVMLAEQAILTRDEASRILHGLAAADERASIDASLRTYLPYEAALKGEIGPVAGKMHIGRSRNDLANAGKRMYLRDQLLRTIEAVIGLRHAVVDKAAGHLDTVMVVYTQRKEAQPITLGHYLMAISENLGKNLDRFRELYPRVNQCPLGAAATAGTGWPLDRDRTADLLGFDGLVVNSIEGVAGWDHVAEFAFDNAIFLSGLSRLASEIQLWSSDEYQMAELDASFAGTSSIMPQKKNPDSLERSRKAAFAAMGPLVGILTSLNGIEYQYSAARVELEPRSIDAMIAATHAMTGVVRTLHPNKEQMLRYAAENYATMTDLTDMLVRRVGIDYREAHEIVARVVMAAIDQGIKANRIGLDLVQQAAIAQTGQPIAVSADDIADALDPVQNVARRKGKGMPAPESVQTAIDDARLELRTDHAWLDSARQRLAAADAALATAVEAIRA

SEQ ID NO: 45 - protein, 495 aa, synthetic construct
MSAHVADATRIGRASGAKAPEFQELYDFDAAALTLTSAVFPYDSKIHRAHVVMLAEQAILTRDEASRILHGLAAADERASIDASLRTYLPYEAALKGEIGPVAGKMHIGRSRNDLANAGKRMFLRDQLLRTIEAVIGLRHAVVDKAAQHLDTVMVVYTQRKEAQPITLGHYLMAISENLGKNLDRFRELYPRVNQCPLGAAATAGTGWPLDRDRTADLLGFDGLVVNSIEGVAGWDHVAEFAFDNAIFLSGLSRLASEIQLWSSDEYQMAELDASFAGTSSIMPQKKNPDSLERSRKAAFAAMGPLVGILTSLNGIEYQYSAARVELEPRSIDAMIAATHAMTGVVRTLHPNKEQMLRYAAENYATMTDLTDMLVRRVGIDYREAHEIVARVVMAAIDQGIKANRIGLDLVQQAAIAQTGQPIAVSADDIADALDPVQNVARRKGKGMPAPESVQTAIDDARLELRTDHAWLDSARQRLAAADAALATAVEAIRA

SEQ ID NO: 46 - protein, 495 aa, synthetic construct
MSAHVADATRIGRASGAKAPEFQELYDFDAAALTLTSAVFPYDSKIHRAHVVMLAEQAILTRDEASRILHGLAAADERASIDASLRTYLPYEAALKGEIGPVAGKMHIGRSRNDLANAGKRMFLRDQLLRTIEAVIGLRHAVVDKAAGHLDTVMVGYTQRKEAQPITLGHYLMAISENLGKNLDRFRELYPRVNQCPLGAAATAGTGWPLDRDRTADLLGFDGLVVNSIEGVAGWDHVAEFAFDNAIFLSGLSRLASEIQLWSSDEYQMAELDASFAGTSSIMPQKKNPDSLERSRKAAFAAMGPLVGILTSLNGIEYQYSAARVELEPRSIDAMIAATHAMTGVVRTLHPNKEQMLRYAAENYATMTDLTDMLVRRVGIDYREAHEIVARVVMAAIDQGIKANRIGLDLVQQAAIAQTGQPIAVSADDIADALDPVQNVARRKGKGMPAPESVQTAIDDARLELRTDHAWLDSARQRLAAADAALATAVEAIRA

SEQ ID NO: 47 - protein, 495 aa, synthetic construct
MSAHVADATRIGRASGAKAPEFQELYDFDAAALTLTSAVFPYDSKIHRAHVVMLAEQAILTRDEASRILHGLAAADERASIDASLRTYLPYEAALKGEIGPVAGKMHIGRSRNDLANAGKRMFLRDQLLRTIEAVIGLRHAVVDKAAGHLDTVMVVYTHRKEAQPITLGHYLMAISENLGKNLDRFRELYPRVNQCPLGAAATAGTGWPLDRDRTADLLGFDGLVVNSIEGVAGWDHVAEFAFDNAIFLSGLSRLASEIQLWSSDEYQMAELDASFAGTSSIMPQKKNPDSLERSRKAAFAAMGPLVGILTSLNGIEYQYSAARVELEPRSIDAMIAATHAMTGVVRTLHPNKEQMLRYAAENYATMTDLTDMLVRRVGIDYREAHEIVARVVMAAIDQGIKANRIGLDLVQQAAIAQTGQPIAVSADDIADALDPVQNVARRKGKGMPAPESVQTAIDDARLELRTDHAWLDSARQRLAAADAALATAVEAIRA

SEQ ID NO: 48 - protein, 495 aa, synthetic construct
MSAHVADATRIGRASGAKAPEFQELYDFDAAALTLTSAVFPYDSKIHRAHVVMLAEQAILTRDEASRILHGLAAADERASIDASLRTYLPYEAALKGEIGPVAGKMHIGRSRNDLANAGKRMFLRDQLLRTIEAVIGLRHAVVDKAAGHLDTVMVVYTQWKEAQPITLGHYLMAISENLGKNLDRFRELYPRVNQCPLGAAATAGTGWPLDRDRTADLLGFDGLVVNSIEGVAGWDHVAEFAFDNAIFLSGLSRLASEIQLWSSDEYQMAELDASFAGTSSIMPQKKNPDSLERSRKAAFAAMGPLVGILTSLNGIEYQYSAARVELEPRSIDAMIAATHAMTGVVRTLHPNKEQMLRYAAENYATMTDLTDMLVRRVGIDYREAHEIVARVVMAAIDQGIKANRIGLDLVQQAAIAQTGQPIAVSADDIADALDPVQNVARRKGKGMPAPESVQTAIDDARLELRTDHAWLDSARQRLAAADAALATAVEAIRA

SEQ ID NO: 49 - protein, 495 aa, synthetic construct
MSAHVADATRIGRASGAKAPEFQELYDFDAAALTLTSAVFPYDSKIHRAHVVMLAEQAILTRDEASRILHGLAAADERASIDASLRTYLPYEAALKGEIGPVAGKMHIGRSRNDLANAGKRMFLRDQLLRTIEAVIGLRHAVVDKAAGHLDTVMVVYTQRREAQPITLGHYLMAISENLGKNLDRFRELYPRVNQCPLGAAATAGTGWPLDRDRTADLLGFDGLVVNSIEGVAGWDHVAEFAFDNAIFLSGLSRLASEIQLWSSDEYQMAELDASFAGTSSIMPQKKNPDSLERSRKAAFAAMGPLVGILTSLNGIEYQYSAARVELEPRSIDAMIAATHAMTGVVRTLHPNKEQMLRYAAENYATMTDLTDMLVRRVGIDYREAHEIVARVVMAAIDQGIKANRIGLDLVQQAAIAQTGQPIAVSADDIADALDPVQNVARRKGKGMPAPESVQTAIDDARLELRTDHAWLDSARQRLAAADAALATAVEAIRA

SEQ ID NO: 50 - protein, 495 aa, synthetic construct
MSAHVADATRIGRASGAKAPEFQELYDFDAAALTLTSAVFPYDSKIHRAHVVMLAEQAILTRDEASRILHGLAAADERASIDASLRTYLPYEAALKGEIGPVAGKMHIGRSRNDLANAGKRMFLRDQLLRTIEAVIGLRHAVVDKAAGHLDTVMVVYTQRKPAQPITLGHYLMAISENLGKNLDRFRELYPRVNQCPLGAAATAGTGWPLDRDRTADLLGFDGLVVNSIEGVAGWDHVAEFAFDNAIFLSGLSRLASEIQLWSSDEYQMAELDASFAGTSSIMPQKKNPDSLERSRKAAFAAMGPLVGILTSLNGIEYQYSAARVELEPRSIDAMIAATHAMTGVVRTLHPNKEQMLRYAAENYATMTDLTDMLVRRVGIDYREAHEIVARVVMAAIDQGIKANRIGLDLVQQAAIAQTGQPIAVSADDIADALDPVQNVARRKGKGMPAPESVQTAIDDARLELRTDHAWLDSARQRLAAADAALATAVEAIRA

SEQ ID NO: 51 - protein, 495 aa, synthetic construct
MSAHVADATRIGRASGAKAPEFQELYDFDAAALTLTSAVFPYDSKIHRAHVVMLAEQAILTRDEASRILHGLAAADERASIDASLRTYLPYEAALKGEIGPVAGKMHIGRSRNDLANAGKRMFLRDQLLRTIEAVIGLRHAVVDKAAGHLDTVMVVYTQRKEAQPITLGHYLMAISENLGRNLDRFRELYPRVNQCPLGAAATAGTGWPLDRDRTADLLGFDGLVVNSIEGVAGWDHVAEFAFDNAIFLSGLSRLASEIQLWSSDEYQMAELDASFAGTSSIMPQKKNPDSLERSRKAAFAAMGPLVGILTSLNGIEYQYSAARVELEPRSIDAMIAATHAMTGVVRTLHPNKEQMLRYAAENYATMTDLTDMLVRRVGIDYREAHEIVARVVMAAIDQGIKANRIGLDLVQQAAIAQTGQPIAVSADDIADALDPVQNVARRKGKGMPAPESVQTAIDDARLELRTDHAWLDSARQRLAAADAALATAVEAIRA

SEQ ID NO: 52 - protein, 495 aa, synthetic construct
MSAHVADATRIGRASGAKAPEFQELYDFDAAALTLTSAVFPYDSKIHRAHVVMLAEQAILTRDEASRILHGLAAADERASIDASLRTYLPYEAALKGEIGPVAGKMHIGRSRNDLANAGKRMFLRDQLLRTIEAVIGLRHAVVDKAAGHLDTVMVVYTQRKEAQPITLGHYLMAISENLGKNLDRFRELYPRVNQCPLGAAATAGTGWPLDRDRTADLLGFDGLVVNSIEGVAGRDHVAEFAFDNAIFLSGLSRLASEIQLWSSDEYQMAELDASFAGTSSIMPQKKNPDSLERSRKAAFAAMGPLVGILTSLNGIEYQYSAARVELEPRSIDAMIAATHAMTGVVRTLHPNKEQMLRYAAENYATMTDLTDMLVRRVGIDYREAHEIVARVVMAAIDQGIKANRIGLDLVQQAAIAQTGQPIAVSADDIADALDPVQNVARRKGKGMPAPESVQTAIDDARLELRTDHAWLDSARQRLAAADAALATAVEAIRA

SEQ ID NO: 53 - protein, 495 aa, synthetic construct
MSAHVADATRIGRASGAKAPEFQELYDFDAAALTLTSAVFPYDSKIHRAHVVMLAEQAILTRDEASRILHGLAAADERASIDASLRTYLPYEAALKGEIGPVAGKMHIGRSRNDLANAGKRMFLRDQLLRTIEAVIGLRHAVVDKAAGHLDTVMVVYTQRKEAQPITLGHYLMAISENLGKNLDRFRELYPRVNQCPLGAAATAGTGWPLDRDRTADLLGFDGLVVNSIEGVAGWDHVAEFAFDNAIFLSGLSRLASEIQLWSSDEYQMAELDASFAGGSSIMPQKKNPDSLERSRKAAFAAMGPLVGILTSLNGIEYQYSAARVELEPRSIDAMIAATHAMTGVVRTLHPNKEQMLRYAAENYATMTDLTDMLVRRVGIDYREAHEIVARVVMAAIDQGIKANRIGLDLVQQAAIAQTGQPIAVSADDIADALDPVQNVARRKGKGMPAPESVQTAIDDARLELRTDHAWLDSARQRLAAADAALATAVEAIRA

SEQ ID NO: 54 - protein, 495 aa, synthetic construct
MSAHVADATRIGRASGAKAPEFQELYDFDAAALTLTSAVFPYDSKIHRAHVVMLAEQAILTRDEASRILHGLAAADERASIDASLRTYLPYEAALKGEIGPVAGKMHIGRSRNDLANAGKRMFLRDQLLRTIEAVIGLRHAVVDKAAGHLDTVMVVYTQRKEAQPITLGHYLMAISENLGKNLDRFRELYPRVNQCPLGAAATAGTGWPLDRDRTADLLGFDGLVVNSIEGVAGWDHVAEFAFDNAIFLSGLSRLASEIQLWSSDEYQMAELDASFAGTSSMMPQKKNPDSLERSRKAAFAAMGPLVGILTSLNGIEYQYSAARVELEPRSIDAMIAATHAMTGVVRTLHPNKEQMLRYAAENYATMTDLTDMLVRRVGIDYREAHEIVARVVMAAIDQGIKANRIGLDLVQQAAIAQTGQPIAVSADDIADALDPVQNVARRKGKGMPAPESVQTAIDDARLELRTDHAWLDSARQRLAAADAALATAVEAIRA

SEQ ID NO: 55 - protein, 495 aa, synthetic construct
MSAHVADATRIGRASGAKAPEFQELYDFDAAALTLTSAVFPYDSKIHRAHVVMLAEQAILTRDEASRILHGLAAADERASIDASLRTYLPYEAALKGEIGPVAGKMHIGRSRNDLANAGKRMFLRDQLLRTIEAVIGLRHAVVDKAAGHLDTVMVVYTQRKEAQPITLGHYLMAISENLGKNLDRFRELYPRVNQCPLGAAATAGTGWPLDRDRTADLLGFDGLVVNSIEGVAGWDHVAEFAFDNAIFLSGLSRLASEIQLWSSDEYQMAELDASFAGTSSIMPQKKNPLSLERSRKAAFAAMGPLVGILTSLNGIEYQYSAARVELEPRSIDAMIAATHAMTGVVRTLHPNKEQMLRYAAENYATMTDLTDMLVRRVGIDYREAHEIVARVVMAAIDQGIKANRIGLDLVQQAAIAQTGQPIAVSADDIADALDPVQNVARRKGKGMPAPESVQTAIDDARLELRTDHAWLDSARQRLAAADAALATAVEAIRA

SEQ ID NO: 56 - protein, 495 aa, synthetic construct
MSAHVADATRIGRASGAKAPEFQELYDFDAAALTLTSAVFPYDSKIHRAHVVMLAEQAILTRDEASRILHGLAAADERASIDASLRTYLPYEAALKGEIGPVAGKMHIGRSRNDLANAGKRMFLRDQLLRTIEAVIGLRHAVVDKAAGHLDTVMVVYTQRKEAQPITLGHYLMAISENLGKNLDRFRELYPRVNQCPLGAAATAGTGWPLDRDRTADLLGFDGLVVNSIEGVAGWDHVAEFAFDNAIFLSGLSRLASEIQLWSSDEYQMAELDASFAGTSSIMPQKKNPDSLELSRKAAFAAMGPLVGILTSLNGIEYQYSAARVELEPRSIDAMIAATHAMTGVVRTLHPNKEQMLRYAAENYATMTDLTDMLVRRVGIDYREAHEIVARVVMAAIDQGIKANRIGLDLVQQAAIAQTGQPIAVSADDIADALDPVQNVARRKGKGMPAPESVQTAIDDARLELRTDHAWLDSARQRLAAADAALATAVEAIRA

SEQ ID NO: 57 - protein, 495 aa, synthetic construct; identical to SEQ ID NO: 56

SEQ ID NO: 58 - protein, 495 aa, synthetic construct
MSAHVADATRIGRASGAKAPEFQELYDFDAAALTLTSAVFPYDSKIHRAHVVMLAEQAILTRDEASRILHGLAAADERASIDASLRTYLPYEAALKGEIGPVAGKMHIGRSRNDLANAGKRMFLRDQLLRTIEAVIGLRHAVVDKAAGHLDTVMVVYTQRKEAQPITLGHYLMAISENLGKNLDRFRELYPRVNQCPLGAAATAGTGWPLDRDRTADLLGFDGLVVNSIEGVAGWDHVAEFAFDNAIFLSGLSRLASEIQLWSSDEYQMAELDASFAGTSSIMPQKKNPDSLERSRGAAFAAMGPLVGILTSLNGIEYQYSAARVELEPRSIDAMIAATHAMTGVVRTLHPNKEQMLRYAAENYATMTDLTDMLVRRVGIDYREAHEIVARVVMAAIDQGIKANRIGLDLVQQAAIAQTGQPIAVSADDIADALDPVQNVARRKGKGMPAPESVQTAIDDARLELRTDHAWLDSARQRLAAADAALATAVEAIRA

SEQ ID NO: 59 - protein, 495 aa, synthetic construct
MSAHVADATRIGRASGAKAPEFQELYDFDAAALTLTSAVFPYDSKIHRAHVVMLAEQAILTRDEASRILHGLAAADERASIDASLRTYLPYEAALKGEIGPVAGKMHIGRSRNDLANAGKRMFLRDQLLRTIEAVIGLRHAVVDKAAGHLDTVMVVYTQRKEAQPITLGHYLMAISENLGKNLDRFRELYPRVNQCPLGAAATAGTGWPLDRDRTADLLGFDGLVVNSIEGVAGWDHVAEFAFDNAIFLSGLSRLASEIQLWSSDEYQMAELDASFAGTSSIMPQKKNPDSLERSRKAAGAAMGPLVGILTSLNGIEYQYSAARVELEPRSIDAMIAATHAMTGVVRTLHPNKEQMLRYAAENYATMTDLTDMLVRRVGIDYREAHEIVARVVMAAIDQGIKANRIGLDLVQQAAIAQTGQPIAVSADDIADALDPVQNVARRKGKGMPAPESVQTAIDDARLELRTDHAWLDSARQRLAAADAALATAVEAIRA

SEQ ID NO: 60 - protein, 495 aa, synthetic construct
MSAHVADATRIGRASGAKAPEFQELYDFDAAALTLTSAVFPYDSKIHRAHVVMLAEQAILTRDEASRILHGLAAADERASIDASLRTYLPYEAALKGEIGPVAGKMHIGRSRNDLANAGKRMFLRDQLLRTIEAVIGLRHAVVDKAAGHLDTVMVVYTQRKEAQPITLGHYLMAISENLGKNLDRFRELYPRVNQCPLGAAATAGTGWPLDRDRTADLLGFDGLVVNSIEGVAGWDHVAEFAFDNAIFLSGLSRLASEIQLWSSDEYQMAELDASFAGTSSIMPQKKNPDSLERSRKAAFAAMGPLVGILTSLNGIPYQYSAARVELEPRSIDAMIAATHAMTGVVRTLHPNKEQMLRYAAENYATMTDLTDMLVRRVGIDYREAHEIVARVVMAAIDQGIKANRIGLDLVQQAAIAQTGQPIAVSADDIADALDPVQNVARRKGKGMPAPESVQTAIDDARLELRTDHAWLDSARQRLAAADAALATAVEAIRA

SEQ ID NO: 61 - protein, 495 aa, synthetic construct
MSAHVADATRIGRASGAKAPEFQELYDFDAAALTLTSAVFPYDSKIHRAHVVMLAEQAILTRDEASRILHGLAAADERASIDASLRTYLPYEAALKGEIGPVAGKMHIGRSRNDLANAGKRMFLRDQLLRTIEAVIGLRHAVVDKAAGHLDTVMVVYTQRKEAQPITLGHYLMAISENLGKNLDRFRELYPRVNQCPLGAAATAGTGWPLDRDRTADLLGFDGLVVNSIEGVAGWDHVAEFAFDNAIFLSGLSRLASEIQLWSSDEYQMAELDASFAGTSSIMPQKKNPDSLERSRKAAFAAMGPLVGILTSLNGIEYTYSAARVELEPRSIDAMIAATHAMTGVVRTLHPNKEQMLRYAAENYATMTDLTDMLVRRVGIDYREAHEIVARVVMAAIDQGIKANRIGLDLVQQAAIAQTGQPIAVSADDIADALDPVQNVARRKGKGMPAPESVQTAIDDARLELRTDHAWLDSARQRLAAADAALATAVEAIRA

SEQ ID NO: 62 - protein, 495 aa, synthetic construct
MSAHVADATRIGRASGAKAPEFQELYDFDAAALTLTSAVFPYDSKIHRAHVVMLAEQAILTRDEASRILHGLAAADERASIDASLRTYLPYEAALKGEIGPVAGKMHIGRSRNDLANAGKRMFLRDQLLRTIEAVIGLRHAVVDKAAGHLDTVMVVYTQRKEAQPITLGHYLMAISENLGKNLDRFRELYPRVNQCPLGAAATAGTGWPLDRDRTADLLGFDGLVVNSIEGVAGWDHVAEFAFDNAIFLSGLSRLASEIQLWSSDEYQMAELDASFAGTSSIMPQKKNPDSLERSRKAAFAAMGPLVGILTSLNGIEYQHSAARVELEPRSIDAMIAATHAMTGVVRTLHPNKEQMLRYAAENYATMTDLTDMLVRRVGIDYREAHEIVARVVMAAIDQGIKANRIGLDLVQQAAIAQTGQPIAVSADDIADALDPVQNVARRKGKGMPAPESVQTAIDDARLELRTDHAWLDSARQRLAAADAALATAVEAIRA

SEQ ID NO: 63 - protein, 495 aa, synthetic construct
MSAHVADATRIGRASGAKAPEFQELYDFDAAALTLTSAVFPYDSKIHRAHVVMLAEQAILTRDEASRILHGLAAADERASIDASLRTYLPYEAALKGEIGPVAGKMHIGRSRNDLANAGKRMFLRDQLLRTIEAVIGLRHAVVDKAAGHLDTVMVVYTQRKEAQPITLGHYLMAISENLGKNLDRFRELYPRVNQCPLGAAATAGTGWPLDRDRTADLLGFDGLVVNSIEGVAGWDHVAEFAFDNAIFLSGLSRLASEIQLWSSDEYQMAELDASFAGTSSIMPQKKNPDSLERSRKAAFAAMGPLVGILTSLNGIEYQYSKARVELEPRSIDAMIAATHAMTGVVRTLHPNKEQMLRYAAENYATMTDLTDMLVRRVGIDYREAHEIVARVVMAAIDQGIKANRIGLDLVQQAAIAQTGQPIAVSADDIADALDPVQNVARRKGKGMPAPESVQTAIDDARLELRTDHAWLDSARQRLAAADAALATAVEAIRA

SEQ ID NO: 64 - protein, 495 aa, synthetic construct
MSAHVADATRIGRASGAKAPEFQELYDFDAAALTLTSAVFPYDSKIHRAHVVMLAEQAILTRDEASRILHGLAAADERASIDASLRTYLPYEAALKGEIGPVAGKMHIGRSRNDLANAGKRMFLRDQLLRTIEAVIGLRHAVVDKAAGHLDTVMVVYTQRKEAQPITLGHYLMAISENLGKNLDRFRELYPRVNQCPLGAAATAGTGWPLDRDRTADLLGFDGLVVNSIEGVAGWDHVAEFAFDNAIFLSGLSRLASEIQLWSSDEYQMAELDASFAGTSSIMPQKKNPDSLERSRKAAFAAMGPLVGILTSLNGIEYQYSADRVELEPRSIDAMIAATHAMTGVVRTLHPNKEQMLRYAAENYATMTDLTDMLVRRVGIDYREAHEIVARVVMAAIDQGIKANRIGLDLVQQAAIAQTGQPIAVSADDIADALDPVQNVARRKGKGMPAPESVQTAIDDARLELRTDHAWLDSARQRLAAADAALATAVEAIRA

SEQ ID NO: 65 - protein, 495 aa, synthetic construct
MSAHVADATRIGRASGAKAPEFQELYDFDAAALTLTSAVFPYDSKIHRAHVVMLAEQAILTRDEASRILHGLAAADERASIDASLRTYLPYEAALKGEIGPVAGKMHIGRSRNDLANAGKRMFLRDQLLRTIEAVIGLRHAVVDKAAGHLDTVMVVYTQRKEAQPITLGHYLMAISENLGKNLDRFRELYPRVNQCPLGAAATAGTGWPLDRDRTADLLGFDGLVVNSIEGVAGWDHVAEFAFDNAIFLSGLSRLASEIQLWSSDEYQMAELDASFAGTSSIMPQKKNPDSLERSRKAAFAAMGPLVGILTSLNGIEYQYSAARQELEPRSIDAMIAATHAMTGVVRTLHPNKEQMLRYAAENYATMTDLTDMLVRRVGIDYREAHEIVARVVMAAIDQGIKANRIGLDLVQQAAIAQTGQPIAVSADDIADALDPVQNVARRKGKGMPAPESVQTAIDDARLELRTDHAWLDSARQRLAAADAALATAVEAIRA

SEQ ID NO: 66 - protein, 495 aa, synthetic construct
MSAHVADATRIGRASGAKAPEFQELYDFDAAALTLTSAVFPYDSKIHRAHVVMLAEQAILTRDEASRILHGLAAADERASIDASLRTYLPYEAALKGEIGPVAGKMHIGRSRNDLANAGKRMFLRDQLLRTIEAVIGLRHAVVDKAAGHLDTVMVVYTQRKEAQPITLGHYLMAISENLGKNLDRFRELYPRVNQCPLGAAATAGTGWPLDRDRTADLLGFDGLVVNSIEGVAGWDHVAEFAFDNAIFLSGLSRLASEIQLWSSDEYQMAELDASFAGTSSIMPQKKNPDSLERSRKAAFAAMGPLVGILTSLNGIEYQYSAARVELEPGSIDAMIAATHAMTGVVRTLHPNKEQMLRYAAENYATMTDLTDMLVRRVGIDYREAHEIVARVVMAAIDQGIKANRIGLDLVQQAAIAQTGQPIAVSADDIADALDPVQNVARRKGKGMPAPESVQTAIDDARLELRTDHAWLDSARQRLAAADAALATAVEAIRA

SEQ ID NO: 67 - protein, 495 aa, synthetic construct
MSAHVADATRIGRASGAKAPEFQELYDFDAAALTLTSAVFPYDSKIHRAHVVMLAEQAILTRDEASRILHGLAAADERASIDASLRTYLPYEAALKGEIGPVAGKMHIGRSRNDLANAGKRMFLRDQLLRTIEAVIGLRHAVVDKAAGHLDTVMVVYTQRKEAQPITLGHYLMAISENLGKNLDRFRELYPRVNQCPLGAAATAGTGWPLDRDRTADLLGFDGLVVNSIEGVAGWDHVAEFAFDNAIFLSGLSRLASEIQLWSSDEYQMAELDASFAGTSSIMPQKKNPDSLERSRKAAFAAMGPLVGILTSLNGIEYQYSAARVELEPRSIDAMIAATHAMTGVVRTLHPNKEQMLRRAAENYATMTDLTDMLVRRVGIDYREAHEIVARVVMAAIDQGIKANRIGLDLVQQAAIAQTGQPIAVSADDIADALDPVQNVARRKGKGMPAPESVQTAIDDARLELRTDHAWLDSARQRLAAADAALATAVEAIRA

SEQ ID NO: 68 - protein, 495 aa, synthetic construct
MSAHVADATRIGRASGAKAPEFQELYDFDAAALTLTSAVFPYDSKIHRAHVVMLAEQAILTRDEASRILHGLAAADERASIDASLRTYLPYEAALKGEIGPVAGKMHIGRSRNDLANAGKRMFLRDQLLRTIEAVIGLRHAVVDKAAGHLDTVMVVYTQRKEAQPITLGHYLMAISENLGKNLDRFRELYPRVNQCPLGAAATAGTGWPLDRDRTADLLGFDGLVVNSIEGVAGWDHVAEFAFDNAIFLSGLSRLASEIQLWSSDEYQMAELDASFAGTSSIMPQKKNPDSLERSRKAAFAAMGPLVGILTSLNGIEYQYSAARVELEPRSIDAMIAATHAMTGVVRTLHPNKEQMLRYAAENYATMTDLADMLVRRVGIDYREAHEIVARVVMAAIDQGIKANRIGLDLVQQAAIAQTGQPIAVSADDIADALDPVQNVARRKGKGMPAPESVQTAIDDARLELRTDHAWLDSARQRLAAADAALATAVEAIRA

SEQ ID NO: 69 - protein, 495 aa, synthetic construct
MSAHVADATRIGRASGAKAPEFQELYDFDAAALTLTSAVFPYDSKIHRAHVVMLAEQAILTRDEASRILHGLAAADERASIDASLRTYLPYEAALKGEIGPVAGKMHIGRSRNDLANAGKRMFLRDQLLRTIEAVIGLRHAVVDKAAGHLDTVMVVYTQRKEAQPITLGHYLMAISENLGKNLDRFRELYPRVNQCPLGAAATAGTGWPLDRDRTADLLGFDGLVVNSIEGVAGWDHVAEFAFDNAIFLSGLSRLASEIQLWSSDEYQMAELDASFAGTSSIMPQKKNPDSLERSRKAAFAAMGPLVGILTSLNGIEYQYSAARVELEPRSIDAMIAATHAMTGVVRTLHPNKEQMLRYAAENYATMTDLTDMLVRRVGIDYREAHEIVARVVRAAIDQGIKANRIGLDLVQQAAIAQTGQPIAVSADDIADALDPVQNVARRKGKGMPAPESVQTAIDDARLELRTDHAWLDSARQRLAAADAALATAVEAIRA

SEQ ID NO: 70 - protein, 495 aa, synthetic construct
MSAHVADATRIGRASGAKAPEFQELYDFDAAALTLTSAVFPYDSKIHRAHVVMLAEQAILTRDEASRILHGLAAADERASIDASLRTYLPYEAALKGEIGPVAGKMHIGRSRNDLANAGKRMFLRDQLLRTIEAVIGLRHAVVDKAAGHLDTVMVVYTQRKEAQPITLGHYLMAISENLGKNLDRFRELYPRVNQCPLGAAATAGTGWPLDRDRTADLLGFDGLVVNSIEGVAGWDHVAEFAFDNAIFLSGLSRLASEIQLWSSDEYQMAELDASFAGTSSIMPQKKNPDSLERSRKAAFAAMGPLVGILTSLNGIEYQYSAARVELEPRSIDAMIAATHAMTGVVRTLHPNKEQMLRYAAENYATMTDLTDMLVRRVGIDYREAHEIVARVVMAAIDQGIKANRIGLDLVQQAAIAQTGQPIAVSADDIADALDPVQNVARRKGKGGPAPESVQTAIDDARLELRTDHAWLDSARQRLAAADAALATAVEAIRA

SEQ ID NO: 71 - DNA, 1488 bp, Chelatococcus asaccharovorans
  source 1..1488: mol_type = other DNA
atgagtgcccatgttgcagatgccacccgtattggccgtgccagtggcgccaaagccccggagttccaggaactgtatgacttcgatgccgccgccctgaccctgaccagtgccgtgttcccgtatgatagtaaaattcatcgcgcccatgtggttatgctggccgaacaggccattctgacccgtgatgaagccagtcgtattctgcatggtctggccgccgcagatgaacgtgccagtattgatgcaagcctgcgtacctatctgccgtatgaagccgccctgaaaggcgaaattggcccggtggcaggtaaaatgcatattggccgtagtcgcaatgatctggcaaatgcaggcaaacgtatgttcctgcgtgatcagctgctgcgcaccattgaagcagttattggtctgcgccatgcagttgttgataaagccgcaggtcatctggataccgtgatggtggtgtatacccagcgtaaagaagcacagccgattaccctgggccattatctgatggccattagcgaaaatctgggtaaaaatctggatcgcttccgtgaactgtatccgcgtgtgaatcagtgtccgctgggcgcagccgcaaccgcaggtacaggttggccgctggatcgtgatcgtaccgcagacttactgggcttcgatggcctggttgtgaatagcattgaaggcgttgcaggctgggatcatgttgccgagttcgccttcgataatgccatcttcctgagcggtctgagtcgtctggccagcgaaattcagctgtggagtagcgatgaatatcagatggcagaactggatgcatcattcgcaggcaccagtagtattatgccgcagaaaaaaaatccggatagcctggaacgtagtcgtaaagcagcattcgcagcaatgggtccgctggttggcattctgaccagcctgaatggcattgaatatcagtatagtgcagcacgtgttgaactggaaccgcgtagtattgatgccatgattgccgccacccatgcaatgaccggcgttgttcgcaccctgcatccgaataaagaacagatgctgcgttatgcagcagaaaattatgcaaccatgaccgatctgaccgatatgctggttcgtcgcgttggcattgattatcgtgaagcacatgaaattgttgcccgcgtggtgatggccgcaattgatcagggtattaaagccaatcgtattggtctggatctggttcagcaggccgcaattgcacagaccggtcagccgattgccgtgagtgcagatgatattgcagatgccctggaccctgttcagaatgttgcccgccgtaaaggcaaaggtatgccggcaccggaaagcgttcagaccgccattgatgatgcacgtctggaactgcgcaccgatcatgcatggctggatagtgcccgccagcgtctggccgccgctgatgcagcactggcaaccgcagtggaagccattcgcgcctaa

SEQ ID NO: 72 - DNA, 1509 bp, Chelativorans sp. BNC1
  source 1..1509: mol_type = other DNA
atgaacatcaacgttccggatgccacccgcattggccgcgccacaggtgcaaaagcaccggagttccaggaactgtatgacttcgatgcagcagcactgaccctgaccagcgccgtgttcccgtatgatagccagattcatcgtgcccatgttgtgatgctgaccgaacagggtattctgaccgtggaagaaagcgccaccattctgagcggcctggcacaggttgatgaactggcagccaccgatggtagcctgcgtacctatctgccgtatgaagcagcactgaaacgcaccattggtagcgtggccggtaaaatgcatattggtcgcagccgcaatgatctggccaatgcaggtaaacgcatgttcctgcgtgatcagctgctgcgtaccattgaagcagttattggctatcgcgaagcagtggttcataaagcagcagatcatctggataccgttatggtggtgtatacccagcgtaaagaagcccagccgattaccctgggtcattatctgatggccattagcgaaaatctggccaaaaatctggatcgttatcgtgaactgtatgcacgtattaatctgtgcccgctgggcgccgcagccaccgcaggtaccggttggcctctgaatcgcgatcgtaccagtgccctgctgggcttcgatggtctggttgtgaatagcattgaaggtgtggcaggttgggatcatgttgccgaacatgcattcgttaatgccgtgttcctgagcggtctgagtcgtctggcaagtgaaattcagctgtggagcaccgatgaatatcaggtggcagaactggatgccagcttcgcaggcaccagcagtattatgccgcagaaaaaaaatccggatagtctggaacgtagccgtaaagccgcattcgccgcaatgggtccgctggttggcattctgaccagtctgaatgcaattgaatatcagtatagcgccgcacgtgttgaactggaaccgcgcagtattgatgccctgattgcagccacccatgcaatgaccggtgtggttcgcaccctgcatccgaataaagaacgcatgcgccagtatgcagcagaaaattatagcaccatgaccgatctgaccgatatgctggttcgtcgcgttggcattgattatcgcgaagcgcatgaaattgtggcccatgtggttattaccgcaattgaaaaaggcattaaagccaataaaatcggtctggatctggtgcaggaagccgccgttgcccagaccggtgcaggtattaatgttagcgccgatgatattaaagatgcactggacccttggcagaatgtgctgcgccgtgaaggtaaaggcatgccggccccgatgagtgtgaaagccagtattgatgatgcaatggcagaactgcataaagatcgtgcctggctggcaaatgcaacccaggcactggcaaatgcgaaacagaccctggcagatagcgtgcagcagattattcagaccgatcgtaaatatctgcgctaa

SEQ ID NO: 73 - DNA, 1830 bp, Bradyrhizobium sp. SK17
  source 1..1830: mol_type = other DNA
atgcgcagcatgattgcagatcgccatccggttagtcatcatattgatagcgcaggtggcgtgtgtccgccgtgcgaaggtcatggcgcagatcgcgccatctggaccgatagtcgtattgcaattgttatgcagccgtgtattaaagcaattgcaccggccggccgcagtcagcatgatccggctgaacatcgcccgagtgttagcgccccgcgtgccgttcgtaatccgattcgccgtgccagtggcccgatgaccctgctgaccgcacgcgcagtgctgaccgcaagttgcagcctggtgctggccgcagccctggcaaccgcaagtacccgcgcccagcagaatccggcactgaatgatggtacccgtattggtcgtagtgcagttccgaaagccccggagttccaggaactgtatgacttcgatgccgccgccaaaaccttaggcgatgcaaccttcccgtatgaagttcgtgtgcatcgcgcccatgtggtgatgctggcagaaaaaggtattgttacccgtagtgatgccgcaaccattctgcgtggcctggataccgtggatgcccgtgccgccgatgatgcaagcctgcgcacctatctgccgtatgaagccgcactgattaaaagcattggtccggttgcaggtcgcatgcataccggccgtagccgcaatgatctggcaaataccgttaatcgcatgttctatcgtgatcagctgaatcgtaccgttgaagcactgattgcactgcgtagtgcagtggttgccaaagcagcagataatctggataccgttatggtggtgtatacccatcgtaaagaagcacagccgattaccctgggtcattatctgatggcaattagtgaaagcctgggcaaaagcattgatcgttatgaacagctgtatgcacgtgtgaatcagagtccgctgggtgccgccgccagcgcaggtaccagttggcctctggatcgcgaacgtaccgcagccctgctgggcttcgatggtctggttattgataccattgaaggtaccgccggctgggatcatattgccgagttcgccagcgataatgcaatctatctgagtggtctgagccgcctggccagcgaaattcagctgtggagcaccgatgaatatcgtagtgccgaactggaccctgcattcgcaggtaccagcagcattatgccgcagaaaaaaaatccggatagcctggaacgtacccgtcagattgcagcaaatagcgttggtgccgttaccagcgttctgaccagcctgaatgcagccgaatatcagcatagtgttacccgtgtgccgctggaaccgcgcagcctggatgccatgattgcagccacccatgccatgaccggcgttgtgcgtaccctgcaaccgaataaagaacagatgctgcgttatgccgcccagaacttcagcaccatgaccgatctggccgataccattgttcgtgaaagcggcattgacttccgtgaagcccatgaaattattgcccgcgttgtggaagccgcaattaatggtggtaaaaccgccgatcagattgatgttgcaatgattgaaaccgcagcccaggcccagctgggtcgcacaattcagattagcgcagccgccgtgcgcgatgcactggaccctgtgcgcagtgttaaactgcgcaatggtattggtggtccggcagccagcagtgtggcagccatgattaaagttagtcaggccgaaattagcgatgaacagagccgcctggcggcccgccgtcaaaaaattgccgcagcaagtgccgcactggcccaggcagttgcagccgctgaacattaa

SEQ ID NO: 74 - DNA, 1488 bp, Brevundimonas diminuta MR-E001
  source 1..1488: mol_type = other DNA
atgaccccgcataatccggatgcaacccgtattggccgtgccagtggcgccaaagccccggaatttcaggaactgtatgattttgaagcagcagcactgaccctgaccagcgcagtttttccgtatgatagtaaaattcatcgtgcccatgttgttatgctggcagaacaggatattctgacccgtgatgaagccgccagtattctgaatggtctggcaaaagccgatgaactggccggtaaagatgcagcactgcgcacctatctgccgtatgaagccgcactgaaacgtgaaattggcagcgttgccggcaaaatgcatattggtcgcagtcgcaatgatctggcaaatgcaggtaaacgtatgtttctgcgtgatcagctgctgcgtaccgttgaagccgttattgcactgcgcgaagcagttgttaccaaagcagccgatcatctggataccgttatggttgtttatacccagcgtaaagaagcacagccgattaccctgggtcattatctgatggcaattagcgaaaatctgggcaaaaatctggcacgttatcgtgaactgcatccgcgtattaatcagtgtccgctgggtgcagcagcaaccgccggcacaggctggcctctggatcgcgatcgtaccgcagcactgctgggttttcatggtctggttgttaatagcattgaaggtgtggccggttgggatcatgttgccgaatttgcatttgataatgccgtgtttctgagtggcctgagtcgcctggccagtgaaattcagctgtggagcaccgatgaatatcagatggccgaactggatagcgcctttgccggtaccagcagcattatgccgcagaaaaaaaatccggatagcctggaacgcagtcgtaaagccgcctttgcagccatgggtccgctggtggccattctgaccagtctgaatggtattgaatatcagtatagcgcagcccgtgttgaactggaaccgcgtagtattgatgcactgattgccgccacccatgcaatgaccggtgttgtgcgtaccctgcatccgaataaagaacagatgctgcgttatgcagccgaaaattatgccaccatgaccgatctgaccgatctgctggtgcgccgcattggtattgattatcgtgaagcccatgaaattgttgcccgcgttgtgatgaccgcaattgaacgcggtattaaagcaaatgccattggcctggatctggtgcaggaagcagccgttgcccagaccggtaatcgcattgaaattggcgccgcagatattgccgatgcactggaccctgtgcagaatgtggcacgtcgcaaaggccgcggcatgccggcacctgaaagtgtgcgcgcagcaattgcagaagcccgccaggaactggatgcagataaagcatggctggaagatcgtcgcgccggcctggccgatgcagatgctgcactggaagaagccgtggccggtattaccacctga

SEQ ID NO: 75 - DNA, 1578 bp, Bradyrhizobium elkanii
  source 1..1578: mol_type = other DNA
atgaccctgctgaccgcacgtgcagttctgaccgcaagctgtagcctggttctggccgcagccctggcaaccgcaagcacccgtgcccagcagaatccggcactgaatgatggtacccgtattggccgtagtgcagtgccgaaagccccggagttccaggaactgtatgacttcgatgcagccgcaaaaaccttaggtgatgcaaccttcccgtatgaagttcgcgtgcatcgcgcacatgtggtgatgctggccgaaaaaggtattgttacccgcagtgatgcagcaaccattctgcgtggtctggataccgttgatgcacgcgccgcagatgatgcaagcctgcgcacctatctgccgtatgaagcagcactgattaaaaccattggtccggtggccggtcgcatgcataccggccgtagtcgtaatgatctggcaaataccgtgaatcgtatgttctatcgcgatcagctgaatcgtaccgtggaagccctgattgcactgcgcagcgccgtggttgcaaaagcagcagataatctggataccgtgatggttgtgtatacccatcgcaaagaagcacagccgattaccctgggccattatctgatggcaattagcgaaagcctgggcaaaagtattgatcgctatgaacagctgtatgcccgtgttaatcagagcccgctgggtgcagcagcaagcgccggtaccagctggccgctggatcgcgaacgtaccgcagccctgctgggcttcgatggcctggttattgataccattgaaggtaccgccggttgggatcatattgcagagttcgccagtgataatgcaatctatctgagcggtctgagtcgtctggcaagtgaaattcagctgtggagtaccgatgaatatcgtagcgccgaactggaccctgccttcgccggcaccagtagcattatgccgcagaaaaaaaatccggatagtctggaacgcacccgtcagattgcagccaatagcgttggtgccgttaccagcgttctgaccagcctgaatgcagccgaatatcagcatagcgtgacccgtgtgccgctggaaccgcgtagcctggatgcaatgattgcagccacccatgcaatgaccggcgtggttcgcaccctgcaaccgaataaagaacagatgctgcgctatgccgcccagaacttcagcaccatgaccgatctggcagataccattgtgcgcgaaagcggtattgacttccgtgaagcacatgaaattattgcacgtgtggtggaagccgcaattaatggcggcaaaaccgcagatcagattgatgttgcaatgattgaaaccgcagcacaggcccagctgggccgtaccattcagattagtgcagccgccgttcgcgatgccctggaccctgttcgcagcgttaaactgcgtaatggcattggtggcccggccgcaagtagtgtggcagcaatgattaaagttagccaggcagaaattagtgatgaacagagccgtctggccgcacgccgccagaaaattgcagccgcaagcgcagcactggcacaggcagtggcagccgccgaacattaa

SEQ ID NO: 76 - DNA, 1557 bp, Pandoraea norimbergensis
  source 1..1557: mol_type = other DNA
atgaaccgcaccccgttcgcactgcgtctggtgaccgccgccgttctgtgtctgagttgggccgcccatgcccagaccccggatgcaagccgcattggtcgcaccagtgttccgaaagccccgggcttccaggcactgtatgacttcgatagcgcagccaaaaccttaccggatgccaccttcccgtatgaagtgcgtgtgcatcgtgcccatgttgtgatgctggccgaaaaaggcattattagccgcgatgatgcacgcaaaattctgaccggcctggataccattgatgcacgtgcacgcgatgatgcgagtctgcgtacctatctgccgtatgaagccgcactggtgaaagaaattggtagcgtggccggtcgcatgcataccggtcgtagtcgtaatgatctggccaataccgtgaatcgcatgttctatcgtgatcagattaatcgtaccgtgaccgccctgattgccctgcgtaccgcagttattgataaagcagaagataatatcgacaccgttatggtggtgtatacccatcgtaaagaagcccagccgattaccctgggccattatctgatggcactgagtgaagcactgaaaaaagatattgatcgttatgaagagctgtatgttcgcatgaatcagagcccgctgggcgccgccgcaagcgcaggtaccggttggcctctggatcgtgaacgtaccgccagtctgctgggcttcgatagtctggttgtggataccattgaaggtaccgcaggttgggatcatattaccgagttcgcagcagataatgccatctatctgagtgatctgggccgcctgggcagcgaaattcagctgtggaccaccgatgaatatcgtctggcagaactggatagcgcctatgccggtattagcagcattatgccgcagaaaaaaaatccggatagcattgaacgtacccgtgccattgcagcaaatagcgtgggtgcactgaccagtattctggttagtctgaatggtattgaatatcagcatagcgtggcccgcgtggccctggaaccgagaagcattgatggcatgattgcagccacccgcgcaatgaccggtgttgttcagagcctgcatgttaataaagcccagatgctgcgtgatgcagccaaaaattatagcaccatgaccgatctggccgatgcaattgtgcgtgatagcggcattgacttccgcgatgcacatgaaattgtggcaaaagttgttgatagcgccattcaggcaaatctgagtgcagatcagattaccgttgatatggtgcgccgtgcagcagaacagcagctgggccataccgttcgtattagcgaagccagtgtgcgtgatgccctggaccctgttcgtaatgttgcccgtcgtgatggcattggtggcccggcaccggcaagcgtgaaacgtatgattgcccaggcacgtaaagaactggatcaggaacaggcacatctgagtcagcgcaccagcgcactgagcagcgcaggtcagcgcctggatgttgcagtggccggtattaccggtaccaattaa

SEQ ID NO: 77 - DNA, 1500 bp, Caballeronia pedi
  source 1..1500: mol_type = other DNA
atgagcaatacccagggtgttaaagatgccacccgcattggtcgcagtagcgttgccaaagccccggagttccaggaactgtatgacttcgatgcagccgcaaaaaccttagttgatgccaccttcccgtatgaaagcgatattcatcatgcccatgtggttatgctggccgaatgtgatattattaaacgcgatgaagcagcacagattctgcgtggcctggaagccgtggatgcacaggcaaaagaaaatccgagcctgcgcacctatctgccgtatgaagccgcactgaaaaaagcagttggcgccgtgggtggtaaaatgcatctgggtcgtagccgcaatgatctggccaatgcagtgaaacgcatgttcctgcgtgatcagctgaatcgtgtgattgaagcagtgattgcactgcgcgcaagtgttgttgccaaagcagccgatcatctggataccgtgatggttgtgtatacccagcgtaaagaagcccagccgattaccctgggtcattatctgatggcatacgctgaaagtctgggcaaaagcctggatcgttatgaacagctgtatgcacgtattaatcagtgcccgctgggtgccgcagccaccgcaggtacaggctggcctctggatcgtgaacgcaccagcgcactgctgggcttcgatagcctggtggttaataccattgaaggtgtggcaggctgggatcatattgccgagttcgcagcagataatgcaatctatatgagtagcctgagtcgtctggcaagcgaaattcagctgtggagcaccgatgaatatcgcagcgcagaactggaccctgccttcgccggtaccagcagtattatgccgcagaaaaaaaatccggatagcctggaacgcacccgccaggccgccttcgctaccatgggccctctggttgccattctgaccagtctgaatggcattgaatatcagtatagcgccgcacgtgttggcctggaaccgcgtagtattgatggtatgattgccgcaacccatgccatgaccggcgttgttcgtaccctgcaaccgaatgccgcacagatgctgcgctatgcagcagaaaacttcgccaccatgaccgatctgaccgatatgctggtgcgcaaaaccggtctggattatcgcgaagcccatgaagttattgcccgtgttgttaatgccgcactggatcagggtaaaaaagccaatgtgattgatctggatctggtgcaggatgccgcacgtgcacagctgggtcataccctggatattagtgcaaccgatgtgcgtgatgccctggaccctgttcagaatgtggcacgccgcaatggtattggtggtccggcaccggttgcagtgcagcgtaccattgataccgcacagcgcgaactggatgaacagcgtgcctgctatgatacccgcatgcgtaaactggcagatgcaagtcgtgaacgtgcccgcgcagttgccagtatgaccgccggcagttaa

SEQ ID NO: 78 - DNA, 1497 bp, Paraburkholderia sartisoli
  source 1..1497: mol_type = other DNA
atgagtgataagcagggtgtggtggatgcaacccgcattggccgcagtagtgttgcaaaagcaccggagttccaggaactgtatgagttcgatgcagcagcaaaaaccttagtggatgcaacattcccgtatgaaagtcagattcatcgtgcccatgtggttatgctggcagaaagcggtattctgaaaacacaagaagtggcagaaattctgcgcggcctggcagtggttgatgaacgtgcccgcagcgatccgagcctgcgtacctatctgccgtatgaagcagccctgaaaaaagtggtgggcagcgttggcggtaaaatgcatctgggccgcagtcgtaatgatctggccaatgcagtgaaacgcatgttcctgcgtgatcaggcaaatcgcaccattgaagccctgattggtctgcgtgcagccgtgattgccaaagcagccgataatctggataccgttatggtggtgtatacccagcgtaaagaagcacagccgattaccctggcacattatctgatggcctatagcgaaggtctgggtaaaagcattgaacgctatgaacagatgtatgcacgtattaatcattgcccgctgggtgccgcagccaccgcaggtacaggctggcctctgaatcgcgaacgtaccagtggcctgctgggcttcgatgcactggttgtgaataccattgaaggtgttgcaggttgggatcatattgccgagttcgccgcaaataatgcaatctatatgagcagcctgagccgtctggcaagtgaaattcagctgtggagtaccgatgaatatcgtgttgccgaactggaccctagcttcgcaggtaccagcagtattatgccgcagaaaaaaaatccggatagtctggaacgtacccgtcaggccgccgccgctgctatgggtccgttcgtgagtattgttaccagcctgaatgccattgaatatcagtatagcgccgcccgtgtgggtctggaaccgcgtagtattgatggcattatggccgcaacccatgccatgaccggcgtggttcgcaccctgcaaccgaataaagcccagatgctgaaatatgccagcgaaaacttcgcaaccatgaccgatctgaccgatatgctggtgcgtgaatgtggcctggattatcgtgaagcccatgaagttattgcccgtgttgtgaatgccgcaattgatgcacgtaaaaccgccaatcagattgatctggatatggtgcaggcagccgcacatgcacagctgggccatccgctggatattagcgcagccgcaattgcagcagcactggaccctgtgcagaatgttggccgtcgtaatggcattggtggcccggcaccgagcagtgtgcagcagatgattgataatgatcgtaaagcactggccgaagaacaggcccgcctggaagatcgcttcgcccgcctgaaacatagtggtaccgatctggatgatgcagttaaacgtattgcaggtctgtaa

SEQ ID NO: 79 - DNA, 1488 bp, synthetic construct
  source 1..1488: mol_type = other DNA
atgaccccgcataatccggatgcaacccgcattggtcgtgcaaaacgcgcaaaagcaccggaatttcaggaactgtatgattttgaagccgcagcactgaccctgaccagcgcagtttttccgtatgatagcaaaattcatcgtgcacatgtggttatgctggcagaacaggatattctgacccgcgatgaagcagcaagcattctgaatggtctggcaaaagcagatgaactggccggcaaagatgccgccctgcgtacctatctgccgtatgaagcagccctgaaacgcgaaattggcagcgttgccggcaaaatgcatattggccgtagtgcaaatgatctgcgcaatcgcgtgaatgcatgcagttgtgttaccgccctgcgtacagttgaagccgttattgccctgcgtgaagcagttgttaccaaagcagccgatcatctggataccgttatggttgtttatacccagcgcaaagaagcccagccgattaccctgggtcattatctgatggcaattagtgaaaatctgggcaaaaatctggcccgctatcgcgaactgcatccgcgcattaatcagtgtccgctgggcgcagccgccaccgcaggtaccggttggcctctggatcgcgatcgtaccgcagccctgctgggttttcatggcctggtggttaatagcattgaaggcgtggcaggctgggatcatgttgcagaatttgcatttgataatgcagtttttctgagtggtctgagtcgcctggccagcgaaattcagctgtggagtaccgatgaatatcagatggcagaactggatagcgcctttgccggcaccagtagcattatgccgcagaaaaaaaatccggatagtctggaacgtagccgcaaaggtgcatttgccgccatgggtccgctggtggcaattctgaccagcctgaatggtattgaatatcagtatagcgccgcccgcgtggaactggaaccgcgtagtattgatgcactgattgccgcaacccatgccatgaccggtgtggtgcgcaccctgcatccgaataaagaacaggatgcatgtgccatgcgtcaggaaaattatgccaccatgaccgatctgaccgatctgctggttcgccgtattggtattgattatcgtgaagcccatgaaattgtggcccgcgttgttatgaccgcaattgaacgtggcattaaagccaatgccattggtctggatctggtgcaggaagccgccgttgcccagaccggtaatcgcattgaaattggtgcagcagatattgccgatgccctggaccctgtgcagaatgtggcacgccgtaaaggtcgtggtatgccggccccggaaagtgttcgtgcagccattgccgaagcccgtcaggaactggatgcagataaagcctggctggaagatcgtcgcgccggcctggcagatgcagatgcagccctggaagaagcagtggccggtattaccacctga

SEQ ID NO: 80 - DNA, 1488 bp, synthetic construct
  source 1..1488: mol_type = other DNA
atgagtgcccatgttgcagatgccacccgtattggccgtgccagtggcgccaaagccccggagttccaggaactgtatgacttcgatgccgccgccctgaccctgaccagtgccgtgttcccgtatgatagtaaaattcatcgcgcccatgtggttatgctggccgaacaggccattctgacccgtgatgaagccagtcgtattctgcatggtctggccgccgcagatgaacgtgccagtattgatgcaagcctgcgtacctatctgccgtatgaagccgccctgaaaggcgaaattggcccggtggcaggtaaaatgcatattggccgtagtcgcaatgatctggcaaatgcaggcaaacgtatgttcctgcgtgatcagctgctgcgcaccattgaagcagttattggtctgcgccatgcagttgttgataaagccgcaggtcatctggataccgtgatggtggtgtatacccagcgtaaagaagcacagccgaccaccctgggccattatctgatggccattagcgaaaatctgggtaaaaatctggatcgcttccgtgaactgtatccgcgtgtgaatcagtgtccgctgggcgcagccgcaaccgcaggtacaggttggccgctggatcgtgatcgtaccgcagacttactgggcttcgatggcctggttgtgaatagcattgaaggcgttgcaggctgggatcatgttgccgagttcgccttcgataatgccatcttcctgagcggtctgagtcgtctggccagcgaaattcagctgtggagtagcgatgaatatcagatggcagaactggatgcatcattcgcaggcaccagtagtattatgccgcagaaaaaaaatccggatagcctggaacgtagtcgtaaagcagcattcgcagcaatgggtccgctggttggcattctgaccagcctgaatggcattgaatatcagtatagtgcagcacgtgttgaactggaaccgcgtagtattgatgccatgattgccgccacccatgcaatgaccggcgttgttcgcaccctgcatccgaataaagaacagatgctgcgttatgcagcagaaaattatgcaaccatgaccgatctgaccgatatgctggttcgtcgcgttggcattgattatcgtgaagcacatgaaattgttgcccgcgtggtgatggccgcaattgatcagggtattaaagccaatcgtattggtctggatctggttcagcaggccgcaattgcacagaccggtcagccgattgccgtgagtgcagatgatattgcagatgccctggaccctgttcagaatgttgcccgccgtaaaggcaaaggtatgccggcaccggaaagcgttcagaccgccattgatgatgcacgtctggaactgcgcaccgatcatgcatggctggatagtgcccgccagcgtctggccgccgctgatgcagcactggcaaccgcagtggaagccattcgcgcctaa

SEQ ID NO: 81 - DNA, 1488 bp, synthetic construct
  source 1..1488: mol_type = other DNA
atgagtgcccatgttgcagatgccacccgtattggccgtgccagtggcgccaaagccccggagttccaggaactgtatgacttcgatgccgccgccctgaccctgaccagtgccgtgttcccgtatgatagtaaaattcatcgcgcccatgtggttatgctggccgaacaggccattctgacccgtgatgaagccagtcgtattctgcatggtctggccgccgcagatgaacgtgccagtattgatgcaagcctgcgtacctatctgccgtatgaagccgccctgaaaggcgaaattggcccggtggcaggtaaaatgcatattggccgtagtcgcaatgatctggcaaatgcaggcgaacgtatgttcctgcgtgatcagctgctgcgcaccattgaagcagttattggtctgcgccatgcagttgttgataaagccgcaggtcatctggataccgtgatggtggtgtatacccagcgtaaagaagcacagccgattaccctgggccattatctgatggccattagcgaaaatctgggtaaaaatctggatcgcttccgtgaactgtatccgcgtgtgaatcagtgtccgctgggcgcagccgcaaccgcaggtacaggttggccgctggatcgtgatcgtaccgcagacttactgggcttcgatggcctggttgtgaatagcattgaaggcgttgcaggctgggatcatgttgccgagttcgccttcgataatgccatcttcctgagcggtctgagtcgtctggccagcgaaattcagctgtggagtagcgatgaatatcagatggcagaactggatgcatcattcgcaggcaccagtagtattatgccgcagaaaaaaaatccggatagcctggaacgtagtcgtaaagcagcattcgcagcaatgggtccgctggttggcattctgaccagcctgaatggcattgaatatcagtatagtgcagcacgtgttgaactggaaccgcgtagtattgatgccatgattgccgccacccatgcaatgaccggcgttgttcgcaccctgcatccgaataaagaacagatgctgcgttatgcagcagaaaattatgcaaccatgaccgatctgaccgatatgctggttcgtcgcgttggcattgattatcgtgaagcacatgaaattgttgcccgcgtggtgatggccgcaattgatcagggtattaaagccaatcgtattggtctggatctggttcagcaggccgcaattgcacagaccggtcagccgattgccgtgagtgcagatgatattgcagatgccctggaccctgttcagaatgttgcccgccgtaaaggcaaaggtatgccggcaccggaaagcgttcagaccgccattgatgatgcacgtctggaactgcgcaccgatcatgcatggctggatagtgcccgccagcgtctggccgccgctgatgcagcactggcaaccgcagtggaagccattcgcgcctaa

SEQ ID NO: 82 - DNA, 1488 bp, synthetic construct
  source 1..1488: mol_type = other DNA
atgagtgcccatgttgcagatgccacccgtattggccgtgccagtggcgccaaagccccggagttccaggaactgtatgacttcgatgccgccgccctgaccctgaccagtgccgtgttcccgtatgatagtaaaattcatcgcgcccatgtggttatgctggccgaacaggccattctgacccgtgatgaagccagtcgtattctgcatggtctggccgccgcagatgaacgtgccagtattgatgcaagcctgcgtacctatctgccgtatgaagccgccctgaaaggcgaaattggcccggtggcaggtaaaatgcatattggccgtagtcgcaatgatctggcaaatgcaggcaaacgtatgttcctgcgtgatcagctgctgcgcaccattgaagcagttattggtctgcgccatgcagttgttgataaagccgcaggtcatctggataccgtgatggtggtgtatacccagcgtaaagaagcacagccgagcaccctgggccattatctgatggccattagcgaaaatctgggtaaaaatctggatcgcttccgtgaactgtatccgcgtgtgaatcagtgtccgctgggcgcagccgcaaccgcaggtacaggttggccgctggatcgtgatcgtaccgcagacttactgggcttcgatggcctggttgtgaatagcattgaaggcgttgcaggctgggatcatgttgccgagttcgccttcgataatgccatcttcctgagcggtctgagtcgtctggccagcgaaattcagctgtggagtagcgatgaatatcagatggcagaactggatgcatcattcgcaggcaccagtagtattatgccgcagaaaaaaaatccggatagcctggaacgtagtcgtaaagcagcattcgcagcaatgggtccgctggttggcattctgaccagcctgaatggcattgaatatcagtatagtgcagcacgtgttgaactggaaccgcgtagtattgatgccatgattgccgccacccatgcaatgaccggcgttgttcgcaccctgcatccgaataaagaacagatgctgcgttatgcagcagaaaattatgcaaccatgaccgatctgaccgatatgctggttcgtcgcgttggcattgattatcgtgaagcacatgaaattgttgcccgcgtggtgatggccgcaattgatcagggtattaaagccaatcgtattggtctggatctggttcagcaggccgcaattgcacagaccggtcagccgattgccgtgagtgcagatgatattgcagatgccctggaccctgttcagaatgttgcccgccgtaaaggcaaaggtatgccggcaccggaaagcgttcagaccgccattgatgatgcacgtctggaactgcgcaccgatcatgcatggctggatagtgcccgccagcgtctggccgccgctgatgcagcactggcaaccgcagtggaagccattcgcgcctaa

SEQ ID NO: 83 - DNA, 1488 bp, synthetic construct
  source 1..1488: mol_type = other DNA
atgagtgcccatgttgcagatgccacccgtattggccgtgccagtggcgccaaagccccggagttccaggaactgtatgacttcgatgccgccgccctgaccctgaccagtgccgtgttcccgtatgatagtaaaattcatcgcgcccatgtggttatgctggccgaacaggccattctgacccgtgatgaagccagtcgtattctgcatggtctggccgccgcagatgaacgtgccagtattgatgcaagcctgcgtacctatctgccgtatgaagccgccctgaaaggcgaaattggcccggtggcaggtaaaatgcatattggccgtagtcgcaatgatctggcaaatgcaggcaaacgtatgttcctgcgtgatcagctgctgcgcaccattgaagcagttattggtctgcgccatgcagttgttgataaagccgcaggtcatctggataccgtgatggtggtgtatacccagcgtaaagaagcacagccgattaccctgggccattatctgatggccattagcgaaaatctgggtaaaaatctggatcgcttccgtgaactgtatccgcgtgtgaatcagtgtccgctgggcgcagccgcaaccgcaggtacaggttggccgctggatcgtgatcgtaccgcagacttactgggcttcgatggcctggttgtgaatagcattgaaggcgttgcaggctgggatcatgttgccgagttcgccttcgataatgccatcttcctgagcggtctgagtcgtctggccagcgaaattcagctgtggagtagcgatgaatatcagatggcagaactggatgcatcattcgcaggcaccagtagtattatgccgcagaaaaaaaatccggatagcctggaacgtagtcgtaaagcagcattcgcagcaatgggtccgctggttggcattctgaccagcctgaatggcattgaatatcagtatagtgcagcacgtgttgaactggaaccgcgtagtattgatgccatgattgccgccacccatgcaatgaccggcgttgttcgcaccctgcatccgaataaagaacagatgctgcgttatgcagcagaaaattatgttaccatgaccgatctgaccgatatgctggttcgtcgcgttggcattgattatcgtgaagcacatgaaattgttgcccgcgtggtgatggccgcaattgatcagggtattaaagccaatcgtattggtctggatctggttcagcaggccgcaattgcacagaccggtcagccgattgccgtgagtgcagatgatattgcagatgccctggaccctgttcagaatgttgcccgccgtaaaggcaaaggtatgccggcaccggaaagcgttcagaccgccattgatgatgcacgtctggaactgcgcaccgatcatgcatggctggatagtgcccgccagcgtctggccgccgctgatgcagcactggcaaccgcagtggaagccattcgcgcctaa

SEQ ID NO: 84 - DNA, 1488 bp, synthetic construct
  source 1..1488: mol_type = other DNA
atgagtgcccatgttgcagatgccacccgtattggccgtgccagtggcgccaaagccccggagttccaggaactgtatgacttcgatgccgccgccctgaccctgaccagtgccgtgttcccgtatgatagtaaaattcatcgcgcccatgtggttatgctggccgaacaggccattctgacccgtgatgaagccagtcgtattctgcatggtctggccgccgcagatgaacgtgccagtattgatgcaagcctgcgtacctatctgccgtatgaagccgccctgaaaggcgaaattggcccggtggcaggtaaaatgcatattggccgtagtcgcaatgatctggcaaatgcaggcgaacgtatgttcctgcgtgatcagctgctgcgcaccattgaagcagttattggtctgcgccatgcagttgttgataaagccgcaggtcatctggataccgtgatggtggtgtatacccagcgtaaagaagcacagccgagcaccctgggccattatctgatggccattagcgaaaatctgggtaaaaatctggatcgcttccgtgaactgtatccgcgtgtgaatcagtgtccgctgggcgcagccgcaaccgcaggtacaggttggccgctggatcgtgatcgtaccgcagacttactgggcttcgatggcctggttgtgaatagcattgaaggcgttgcaggctgggatcatgttgccgagttcgccttcgataatgccatcttcctgagcggtctgagtcgtctggccagcgaaattcagctgtggagtagcgatgaatatcagatggcagaactggatgcatcattcgcaggcaccagtagtattatgccgcagaaaaaaaatccggatagcctggaacgtagtcgtaaagcagcattcgcagcaatgggtccgctggttggcattctgaccagcctgaatggcattgaatatcagtatagtgcagcacgtgttgaactggaaccgcgtagtattgatgccatgattgccgccacccatgcaatgaccggcgttgttcgcaccctgcatccgaataaagaacagatgctgcgttatgcagcagaaaattatgttaccatgaccgatctgaccgatatgctggttcgtcgcgttggcattgattatcgtgaagcacatgaaattgttgcccgcgtggtgatggccgcaattgatcagggtattaaagccaatcgtattggtctggatctggttcagcaggccgcaattgcacagaccggtcagccgattgccgtgagtgcagatgatattgcagatgccctggaccctgttcagaatgttgcccgccgtaaaggcaaaggtatgccggcaccggaaagcgttcagaccgccattgatgatgcacgtctggaactgcgcaccgatcatgcatggctggatagtgcccgccagcgtctggccgccgctgatgcagcactggcaaccgcagtggaagccattcgcgcctaa

SEQ ID NO: 85 - DNA, 1488 bp, synthetic construct
  source 1..1488: mol_type = other DNA
atgagtgcccatgttgcagatgccacccgtattggccgtgccagtggcgccaaagccccggagttccaggaactgtatgacttcgatgccgccgccctgaccctgaccagtgccgtgttcccgtatgatagtaaaattcatcgcgcccatgtggttatgctggccgaacaggccattctgacccgtgatgaagccagtcgtattctgcatggtctggccgccgcagatgaacgtgccagtattgatgcaagcctgcgtacctatctgccgtatgaagccgccctgaaaggcgaaattggcccggtggcaggtaaaatgcatattggccgtagtcgcaatgatctggcaaatgcaggcgaacgtatgttcctgcgtgatcagctgctgcgcaccattgaagcagttattggtctgcgccatgcagttgttgataaagccgcaggtcatctggataccgtgatggtggtgtatacccagcgtaaagaagcacagccgaccaccctgggccattatctgatggccattagcgaaaatctgggtaaaaatctggatcgcttccgtgaactgtatccgcgtgtgaatcagtgtccgctgggcgcagccgcaaccgcaggtacaggttggccgctggatcgtgatcgtaccgcagacttactgggcttcgatggcctggttgtgaatagcattgaaggcgttgcaggctgggatcatgttgccgagttcgccttcgataatgccatcttcctgagcggtctgagtcgtctggccagcgaaattcagctgtggagtagcgatgaatatcagatggcagaactggatgcatcattcgcaggcaccagtagtattatgccgcagaaaaaaaatccggatagcctggaacgtagtcgtaaagcagcattcgcagcaatgggtccgctggttggcattctgaccagcctgaatggcattgaatatcagtatagtgcagcacgtgttgaactggaaccgcgtagtattgatgccatgattgccgccacccatgcaatgaccggcgttgttcgcaccctgcatccgaataaagaacagatgctgcgttatgcagcagaaaattatgttaccatgaccgatctgaccgatatgctggttcgtcgcgttggcattgattatcgtgaagcacatgaaattgttgcccgcgtggtgatggccgcaattgatcagggtattaaagccaatcgtattggtctggatctggttcagcaggccgcaattgcacagaccggtcagccgattgccgtgagtgcagatgatattgcagatgccctggaccctgttcagaatgttgcccgccgtaaaggcaaaggtatgccggcaccggaaagcgttcagaccgccattgatgatgcacgtctggaactgcgcaccgatcatgcatggctggatagtgcccgccagcgtctggccgccgctgatgcagcactggcaaccgcagtggaagccattcgcgcctaa

SEQ ID NO: 86 - DNA, 1509 bp, synthetic construct
  source 1..1509: mol_type = other DNA
atgaacatcaacgttccggatgccacccgcattggccgcgccacaggtgcaaaagcaccggagttccaggaactgtatgacttcgatgcagcagcactgaccctgaccagcgccgtgttcccgtatgatagccagattcatcgtgcccatgttgtgatgctgaccgaacagggtattctgaccgtggaagaaagcgccaccattctgagcggcctggcacaggttgatgaactggcagccaccgatggtagcctgcgtacctatctgccgtatgaagcagcactgaaacgcaccattggtagcgtggccggtaaaatgcatattggtcgcagccgcaatgatctggccaatgcaggtaaacgcatgttcctgcgtgatcagctgctgcgtaccattgaagcagttattggctatcgcgaagcagtggttcataaagcagcagatcatctggataccgttatggtggtgtatacccagcgtaaagaagcccagccgagcaccctgggtcattatctgatggccattagcgaaaatctggccaaaaatctggatcgttatcgtgaactgtatgcacgtattaatctgtgcccgctgggcgccgcagccaccgcaggtaccggttggcctctgaatcgcgatcgtaccagtgccctgctgggcttcgatggtctggttgtgaatagcattgaaggtgtggcaggttgggatcatgttgccgaacatgcattcgttaatgccgtgttcctgagcggtctgagtcgtctggcaagtgaaattcagctgtggagcaccgatgaatatcaggtggcagaactggatgccagcttcgcaggcaccagcagtattatgccgcagaaaaaaaatccggatagtctggaacgtagccgtaaagccgcattcgccgcaatgggtccgctggttggcattctgaccagtctgaatgcaattgaatatcagtatagcgccgcacgtgttgaactggaaccgcgcagtattgatgccctgattgcagccacccatgcaatgaccggtgtggttcgcaccctgcatccgaataaagaacgcatgcgccagtatgcagcagaaaattatagcaccatgaccgatctgaccgatatgctggttcgtcgcgttggcattgattatcgcgaagcgcatgaaattgtggcccatgtggttattaccgcaattgaaaaaggcattaaagccaataaaatcggtctggatctggtgcaggaagccgccgttgcccagaccggtgcaggtattaatgttagcgccgatgatattaaagatgcactggacccttggcagaatgtgctgcgccgtgaaggtaaaggcatgccggccccgatgagtgtgaaagccagtattgatgatgcaatggcagaactgcataaagatcgtgcctggctggcaaatgcaacccaggcactggcaaatgcgaaacagaccctggcagatagcgtgcagcagattattcagaccgatcgtaaatatctgcgctaa

SEQ ID NO: 87 - DNA, 1509 bp, synthetic construct
  source 1..1509: mol_type = other DNA
atgaacatcaacgttccggatgccacccgcattggccgcgccacaggtgcaaaagcaccggagttccaggaactgtatgacttcgatgcagcagcactgaccctgaccagcgccgtgttcccgtatgatagccagattcatcgtgcccatgttgtgatgctgaccgaacagggtattctgaccgtggaagaaagcgccaccattctgagcggcctggcacaggttgatgaactggcagccaccgatggtagcctgcgtacctatctgccgtatgaagcagcactgaaacgcaccattggtagcgtggccggtaaaatgcatattggtcgcagccgcaatgatctggccaatgcaggtgaacgcatgttcctgcgtgatcagctgctgcgtaccattgaagcagttattggctatcgcgaagcagtggttcataaagcagcagatcatctggataccgttatggtggtgtatacccagcgtaaagaagcccagccgagcaccctgggtcattatctgatggccattagcgaaaatctggccaaaaatctggatcgttatcgtgaactgtatgcacgtattaatctgtgcccgctgggcgccgcagccaccgcaggtaccggttggcctctgaatcgcgatcgtaccagtgccctgctgggcttcgatggtctggttgtgaatagcattgaaggtgtggcaggttgggatcatgttgccgaacatgcattcgttaatgccgtgttcctgagcggtctgagtcgtctggcaagtgaaattcagctgtggagcaccgatgaatatcaggtggcagaactggatgccagcttcgcaggcaccagcagtattatgccgcagaaaaaaaatccggatagtctggaacgtagccgtaaagccgcattcgccgcaatgggtccgctggttggcattctgaccagtctgaatgcaattgaatatcagtatagcgccgcacgtgttgaactggaaccgcgcagtattgatgccctgattgcagccacccatgcaatgaccggtgtggttcgcaccctgcatccgaataaagaacgcatgcgccagtatgcagcagaaaattatgttaccatgaccgatctgaccgatatgctggttcgtcgcgttggcattgattatcgcgaagcgcatgaaattgtggcccatgtggttattaccgcaattgaaaaaggcattaaagccaataaaatcggtctggatctggtgcaggaagccgccgttgcccagaccggtgcaggtattaatgttagcgccgatgatattaaagatgcactggacccttggcagaatgtgctgcgccgtgaaggtaaaggcatgccggccccgatgagtgtgaaagccagtattgatgatgcaatggcagaactgcataaagatcgtgcctggctggcaaatgcaacccaggcactggcaaatgcgaaacagaccctggcagatagcgtgcagcagattattcagaccgatcgtaaatatctgcgctaa

SEQ ID NO: 88 - DNA, 1509 bp, synthetic construct
  source 1..1509: mol_type = other DNA
atgaacatcaacgttccggatgccacccgcattggccgcgccacaggtgcaaaagcaccggagttccaggaactgtatgacttcgatgcagcagcactgaccctgaccagcgccgtgttcccgtatgatagccagattcatcgtgcccatgttgtgatgctgaccgaacagggtattctgaccgtggaagaaagcgccaccattctgagcggcctggcacaggttgatgaactggcagccaccgatggtagcctgcgtacctatctgccgtatgaagcagcactgaaacgcaccattggtagcgtggccggtaaaatgcatattggtcgcagccgcaatgatctggccaatgcaggtaaacgcatgttcctgcgtgatcagctgctgcgtaccattgaagcagttattggctatcgcgaagcagtggttcataaagcagcagatcatctggataccgttatggtggtgtatacccagcgtaaagaagcccagccgattaccctgggtcattatctgatggccattagcgaaaatctggccaaaaatctggatcgttatcgtgaactgtatgcacgtattaatctgtgcccgctgggcgccgcagccaccgcaggtaccggttggcctctgaatcgcgatcgtaccagtgccctgctgggcttcgatggtctggttgtgaatagcattgaaggtgtggcaggttgggatcatgttgccgaacatgcattcgttaatgccgtgttcctgagcggtctgagtcgtctggcaagtgaaattcagctgtggagcaccgatgaatatcaggtggcagaactggatgccagcttcgcaggcaccagcagtattatgccgcagaaaaaaaatccggatagtctggaacgtagccgtaaagccgcattcgccgcaatgggtccgctggttggcattctgaccagtctgaatgcaattgaatatcagtatagcgccgcacgtgttgaactggaaccgcgcagtattgatgccctgattgcagccacccatgcaatgaccggtgtggttcgcaccctgcatccgaataaagaacgcatgcgccagtatgcagcagaaaattatgttaccatgaccgatctgaccgatatgctggttcgtcgcgttggcattgattatcgcgaagcgcatgaaattgtggcccatgtggttattaccgcaattgaaaaaggcattaaagccaataaaatcggtctggatctggtgcaggaagccgccgttgcccagaccggtgcaggtattaatgttagcgccgatgatattaaagatgcactggacccttggcagaatgtgctgcgccgtgaaggtaaaggcatgccggccccgatgagtgtgaaagccagtattgatgatgcaatggcagaactgcataaagatcgtgcctggctggcaaatgcaacccaggcactggcaaatgcgaaacagaccctggcagatagcgtgcagcagattattcagaccgatcgtaaatatctgcgctaa

SEQ ID NO: 89 - DNA, 1509 bp, synthetic construct
  source 1..1509: mol_type = other DNA
atgaacatcaacgttccggatgccacccgcattggccgcgccacaggtgcaaaagcaccggagttccaggaactgtatgacttcgatgcagcagcactgaccctgaccagcgccgtgttcccgtatgatagccagattcatcgtgcccatgttgtgatgctgaccgaacagggtattctgaccgtggaagaaagcgccaccattctgagcggcctggcacaggttgatgaactggcagccaccgatggtagcctgcgtacctatctgccgtatgaagcagcactgaaacgcaccattggtagcgtggccggtaaaatgcatattggtcgcagccgcaatgatctggccaatgcaggtgaacgcatgttcctgcgtgatcagctgctgcgtaccattgaagcagttattggctatcgcgaagcagtggttcataaagcagcagatcatctggataccgttatggtggtgtatacccagcgtaaagaagcccagccgaccaccctgggtcattatctgatggccattagcgaaaatctggccaaaaatctggatcgttatcgtgaactgtatgcacgtattaatctgtgcccgctgggcgccgcagccaccgcaggtaccggttggcctctgaatcgcgatcgtaccagtgccctgctgggcttcgatggtctggttgtgaatagcattgaaggtgtggcaggttgggatcatgttgccgaacatgcattcgttaatgccgtgttcctgagcggtctgagtcgtctggcaagtgaaattcagctgtggagcaccgatgaatatcaggtggcagaactggatgccagcttcgcaggcaccagcagtattatgccgcagaaaaaaaatccggatagtctggaacgtagccgtaaagccgcattcgccgcaatgggtccgctggttggcattctgaccagtctgaatgcaattgaatatcagtatagcgccgcacgtgttgaactggaaccgcgcagtattgatgccctgattgcagccacccatgcaatgaccggtgtggttcgcaccctgcatccgaataaagaacgcatgcgccagtatgcagcagaaaattatgttaccatgaccgatctgaccgatatgctggttcgtcgcgttggcattgattatcgcgaagcgcatgaaattgtggcccatgtggttattaccgcaattgaaaaaggcattaaagccaataaaatcggtctggatctggtgcaggaagccgccgttgcccagaccggtgcaggtattaatgttagcgccgatgatattaaagatgcactggacccttggcagaatgtgctgcgccgtgaaggtaaaggcatgccggccccgatgagtgtgaaagccagtattgatgatgcaatggcagaactgcataaagatcgtgcctggctggcaaatgcaacccaggcactggcaaatgcgaaacagaccctggcagatagcgtgcagcagattattcagaccgatcgtaaatatctgcgctaa

SEQ ID NO: 90 - DNA, 1509 bp, synthetic construct
  source 1..1509: mol_type = other DNA
atgaacatcaacgttccggatgccacccgcattggccgcgccacaggtgcaaaagcaccggagttccaggaactgtatgacttcgatgcagcagcactgaccctgaccagcgccgtgttcccgtatgatagccagattcatcgtgcccatgttgtgatgctgaccgaacagggtattctgaccgtggaagaaagcgccaccattctgagcggcctggcacaggttgatgaactggcagccaccgatggtagcctgcgtacctatctgccgtatgaagcagcactgaaacgcaccattggtagcgtggccggtaaaatgcatattggtcgcagccgcaatgatctggccaatgcaggtgaacgcatgttcctgcgtgatcagctgctgcgtaccattgaagcagttattggctatcgcgaagcagtggttcataaagcagcagatcatctggataccgttatggtggtgtatacccagcgtaaagaagcccagccgattaccctgggtcattatctgatggccattagcgaaaatctggccaaaaatctggatcgttatcgtgaactgtatgcacgtattaatctgtgcccgctgggcgccgcagccaccgcaggtaccggttggcctctgaatcgcgatcgtaccagtgccctgctgggcttcgatggtctggttgtgaatagcattgaaggtgtggcaggttgggatcatgttgccgaacatgcattcgttaatgccgtgttcctgagcggtctgagtcgtctggcaagtgaaattcagctgtggagcaccgatgaatatcaggtggcagaactggatgccagcttcgcaggcaccagcagtattatgccgcagaaaaaaaatccggatagtctggaacgtagccgtaaagccgcattcgccgcaatgggtccgctggttggcattctgaccagtctgaatgcaattgaatatcagtatagcgccgcacgtgttgaactggaaccgcgcagtattgatgccctgattgcagccacccatgcaatgaccggtgtggttcgcaccctgcatccgaataaagaacgcatgcgccagtatgcagcagaaaattatagcaccatgaccgatctgaccgatatgctggttcgtcgcgttggcattgattatcgcgaagcgcatgaaattgtggcccatgtggttattaccgcaattgaaaaaggcattaaagccaataaaatcggtctggatctggtgcaggaagccgccgttgcccagaccggtgcaggtattaatgttagcgccgatgatattaaagatgcactggacccttggcagaatgtgctgcgccgtgaaggtaaaggcatgccggccccgatgagtgtgaaagccagtattgatgatgcaatggcagaactgcataaagatcgtgcctggctggcaaatgcaacccaggcactggcaaatgcgaaacagaccctggcagatagcgtgcagcagattattcagaccgatcgtaaatatctgcgctaa

SEQ ID NO: 91 - DNA, 1509 bp, synthetic construct
  source 1..1509: mol_type = other DNA
atgaacatcaacgttccggatgccacccgcattggccgcgccacaggtgcaaaagcaccggagttccaggaactgtatgacttcgatgcagcagcactgaccctgaccagcgccgtgttcccgtatgatagccagattcatcgtgcccatgttgtgatgctgaccgaacagggtattctgaccgtggaagaaagcgccaccattctgagcggcctggcacaggttgatgaactggcagccaccgatggtagcctgcgtacctatctgccgtatgaagcagcactgaaacgcaccattggtagcgtggccggtaaaatgcatattggtcgcagccgcaatgatctggccaatgcaggtaaacgcatgttcctgcgtgatcagctgctgcgtaccattgaagcagttattggctatcgcgaagcagtggttcataaagcagcagatcatctggataccgttatggtggtgtatacccagcgtaaagaagcccagccgaccaccctgggtcattatctgatggccattagcgaaaatctggccaaaaatctggatcgttatcgtgaactgtatgcacgtattaatctgtgcccgctgggcgccgcagccaccgcaggtaccggttggcctctgaatcgcgatcgtaccagtgccctgctgggcttcgatggtctggttgtgaatagcattgaaggtgtggcaggttgggatcatgttgccgaacatgcattcgttaatgccgtgttcctgagcggtctgagtcgtctggcaagtgaaattcagctgtggagcaccgatgaatatcaggtggcagaactggatgccagcttcgcaggcaccagcagtattatgccgcagaaaaaaaatccggatagtctggaacgtagccgtaaagccgcattcgccgcaatgggtccgctggttggcattctgaccagtctgaatgcaattgaatatcagtatagcgccgcacgtgttgaactggaaccgcgcagtattgatgccctgattgcagccacccatgcaatgaccggtgtggttcgcaccctgcatccgaataaagaacgcatgcgccagtatgcagcagaaaattatagcaccatgaccgatctgaccgatatgctggttcgtcgcgttggcattgattatcgcgaagcgcatgaaattgtggcccatgtggttattaccgcaattgaaaaaggcattaaagccaataaaatcggtctggatctggtgcaggaagccgccgttgcccagaccggtgcaggtattaatgttagcgccgatgatattaaagatgcactggacccttggcagaatgtgctgcgccgtgaaggtaaaggcatgccggccccgatgagtgtgaaagccagtattgatgatgcaatggcagaactgcataaagatcgtgcctggctggcaaatgcaacccaggcactggcaaatgcgaaacagaccctggcagatagcgtgcagcagattattcagaccgatcgtaaatatctgcgctaa